European Patent Application EP 4 768 503 A1, published July 1, 2026. Title: 阿尔茨海默病治疗剂的开发和应用. Applicant: 康诺亚生物医药科技（成都）有限公司. The sequence listing filed with the application follows.

SEQUENCE LISTING (280 sequences)

SEQ ID NO: 1 - protein, 124 aa, synthetic construct
  REGION 1..124: note = 192E15 VH
EVKLVESGGGLVQPGGSRKLSCAASGFTFSDYGMAWVRQAPGKGPEWVAFISNLAYSIYYADTVTGRFTISRQNAKNTLYLEMSSLRSEDTAMYYCARDRGYDGHSPYYAMDYWGQGTSVTVSS

SEQ ID NO: 2 - DNA, 372 bp, synthetic construct
  misc_feature 1..372: note = Nucleotide sequence of 192E15 VH
  source 1..372: mol_type = other DNA
gaggtgaagctggtggagtctgggggaggcttagtgcagcctggagggtcccggaaactctcctgtgcagcctctggattcactttcagtgactacggaatggcgtgggttcgacaggctccagggaaggggcctgagtgggtggcattcattagtaatttggcatatagtatttactatgcagacactgtgacgggccgattcaccatctctagacagaatgccaagaacaccctgtacctggaaatgagcagtctgaggtctgaggacacagccatgtactactgtgcaagggatcgggggtatgatggtcactccccttactatgctatggactactggggtcagggaacctcagtcaccgtctcctca

SEQ ID NO: 3 - protein, 5 aa, synthetic construct
  REGION 1..5: note = 192E15, 156N21 HCDR1
DYGMA

SEQ ID NO: 4 - protein, 17 aa, synthetic construct
  REGION 1..17: note = 192E15, 156N21 HCDR2
FISNLAYSIYYADTVTG

SEQ ID NO: 5 - protein, 15 aa, synthetic construct
  REGION 1..15: note = 192E15 HCDR3
DRGYDGHSPYYAMDY

SEQ ID NO: 6 - protein, 109 aa, synthetic construct
  REGION 1..109: note = 192E15 VL
QAVVTQESALTTSPGETVTLTCRSSTGAVTTSNYANWVQEKPDHLFTGLIGGTSNRPPGVPARFSGSLIGDKAALTITGAQTEDEAIYFCALWYSHHWVFGGGTKLTVL

SEQ ID NO: 7 - DNA, 327 bp, synthetic construct
  misc_feature 1..327: note = Nucleotide sequence of 192E15 VL
  source 1..327: mol_type = other DNA
caggctgttgtgactcaggaatctgcactcaccacatcacctggtgaaacagtcacactcacttgtcgctcaagtactggggctgttacaactagtaactatgccaactgggtccaagaaaaaccagatcatttattcactggtctaattggtggtaccagcaaccgacctccaggtgttcctgccagattctcaggctccctgattggagacaaggctgccctcaccatcacaggggcacagactgaggatgaggcaatatatttctgtgctctatggtacagccaccactgggtgttcggtggaggaaccaaactgactgtccta

SEQ ID NO: 8 - protein, 14 aa, synthetic construct
  REGION 1..14: note = 192E15 LCDR1
RSSTGAVTTSNYAN

SEQ ID NO: 9 - protein, 7 aa, synthetic construct
  REGION 1..7: note = 192E15 LCDR2
GTSNRPP

SEQ ID NO: 10 - protein, 9 aa, synthetic construct
  REGION 1..9: note = 192E15 LCDR3
ALWYSHHWV

SEQ ID NO: 11 - protein, 126 aa, synthetic construct
  REGION 1..126: note = 179M22 VH
EVMLVESGRDLVKPGGSLKLSCAASGFTFSAYAMSWVRQTPEKRLEWVATITSRGTYTYYPDSVKGRFTISRDNAKNTLYLQMHSLRSEDTAMYYCVRHELITTVVSTDYFSLDYWGQGTSVTVSS

SEQ ID NO: 12 - DNA, 378 bp, synthetic construct
  misc_feature 1..378: note = Nucleotide sequence of 179M22 VH
  source 1..378: mol_type = other DNA
gaagtgatgctggtggagtctgggagagacttagtgaagcctggagggtccctgaaactctcctgtgcagcctctggattcactttcagtgcctatgccatgtcttgggttcgccagactccggagaagaggctggagtgggtcgcaaccattactagtcgtggtacttacacctactatccagacagtgtgaaggggcgattcaccatctccagagacaatgccaagaacaccctgtacctgcaaatgcacagtctgaggtctgaggacacggccatgtattactgtgtgagacatgagcttattactacggtagtatctacggattacttttctctggactactggggtcaaggaacctcagtcaccgtctcctca

SEQ ID NO: 13 - protein, 5 aa, synthetic construct
  REGION 1..5: note = 179M22 HCDR1
AYAMS

SEQ ID NO: 14 - protein, 17 aa, synthetic construct
  REGION 1..17: note = 179M22 HCDR2
TITSRGTYTYYPDSVKG

SEQ ID NO: 15 - protein, 17 aa, synthetic construct
  REGION 1..17: note = 179M22 HCDR3
HELITTVVSTDYFSLDY

SEQ ID NO: 16 - protein, 111 aa, synthetic construct
  REGION 1..111: note = 179M22 VL
DIVLTQSPASLAVSLGQRATISCRASDSVEYYGTSLMQWYQQKPGQPPKLLIYAASNVESGVPARFSGSGSGTDFSLNIHPVEEDDVAMYFCQQSRKVPLTFGAGTKLELK

SEQ ID NO: 17 - DNA, 333 bp, synthetic construct
  misc_feature 1..333: note = Nucleotide sequence of 179M22 VL
  source 1..333: mol_type = other DNA
gacattgtgctcacccaatctccagcttctttggctgtgtccctagggcagagagccaccatctcctgtagagccagtgacagtgttgaatattatggcacaagtttaatgcagtggtaccaacagaaaccaggacagccacccaaactcctcatctatgctgcatccaacgtagaatctggggtccctgccaggtttagtggcagtgggtctgggacagacttcagcctcaacatccatcctgtggaggaggatgatgttgcaatgtatttctgtcagcaaagtaggaaggttccgctcacgttcggtgctgggaccaagctggagctgaaa

SEQ ID NO: 18 - protein, 15 aa, synthetic construct
  REGION 1..15: note = 179M22 LCDR1
RASDSVEYYGTSLMQ

SEQ ID NO: 19 - protein, 7 aa, synthetic construct
  REGION 1..7: note = 179M22, 175P19, 185O18 LCDR2
AASNVES

SEQ ID NO: 20 - protein, 9 aa, synthetic construct
  REGION 1..9: note = 179M22, 175P19, 185O18 LCDR3
QQSRKVPLT

SEQ ID NO: 21 - protein, 117 aa, synthetic construct
  REGION 1..117: note = 200O1 VH
QVQLKESGPGLVAPSQSLSITCTVSGFSLSRYIVHWYRQPPGKGLEWLGMIWGGGRIDYNSALKSRLSISKDNSKSQVFLKMNSLQTDDTAMYYCARNFGENAEAYWGQGTLVTVSA

SEQ ID NO: 22 - DNA, 351 bp, synthetic construct
  misc_feature 1..351: note = Nucleotide sequence of 200O1 VH
  source 1..351: mol_type = other DNA
caggtgcaactgaaggagtcaggacctggcctggtggcaccctcacagagcctgtccatcacatgcactgtctctgggttctcattatccagatatattgtacactggtatcggcagcctccaggaaagggtctggagtggctgggaatgatatggggtggtggaaggatagactataattcagctctcaaatccagactgagcatcagtaaggacaactccaagagccaagtttttttaaaaatgaacagtctgcaaactgatgacacagccatgtactactgtgccagaaatttcggggaaaacgccgaggcttattggggccaagggactctggtcactgtctctgca

SEQ ID NO: 23 - protein, 5 aa, synthetic construct
  REGION 1..5: note = 200O1, h200O1 H1, h200O1 H2, h200O1 H3, h200O1 H4, h200O1 H5,h200O1 H6, h200O1 H7, h200O1 H8, h200O1 H9 HCDR1
RYIVH

SEQ ID NO: 24 - protein, 16 aa, synthetic construct
  REGION 1..16: note = 200O1, h200O1 H1, h200O1 H2, h200O1 H5, h200O1 H6 HCDR2
MIWGGGRIDYNSALKS

SEQ ID NO: 25 - protein, 9 aa, synthetic construct
  REGION 1..9: note = 200O1, h200O1 H1, h200O1 H2, h200O1 H3, h200O1 H4, h200O1 H5,h200O1 H6, h200O1 H7, h200O1 H8, h200O1 H9 HCDR3
NFGENAEAY

SEQ ID NO: 26 - protein, 107 aa, synthetic construct
  REGION 1..107: note = 200O1 VL
DIQMTQTTSSLSASLGDRVTITCRASQDINIYLNWYQQKPDGVVKLLIYYTSRLHSGVPSRFSGSGSGTDFSLTISNLEQEDIATYFCQQGHTLPYTFGGGTKLEIK

SEQ ID NO: 27 - DNA, 321 bp, synthetic construct
  misc_feature 1..321: note = Nucleotide sequence of 200O1 VL
  source 1..321: mol_type = other DNA
gatatccagatgacacagactacatcctccctgtctgcctctctgggagacagagtcaccatcacttgcagggcaagtcaggacattaacatttatttaaactggtatcagcagaaaccagatggagttgttaaactcctgatctactacacatcaagattacattcaggagtcccatcaaggttcagtggcagtgggtctggaacagatttttctctcaccattagcaacctggagcaagaagatattgccacttacttttgccaacagggtcatacacttccgtacacgttcggaggggggaccaagctggaaataaaa

SEQ ID NO: 28 - protein, 11 aa, synthetic construct
  REGION 1..11: note = 200O1, h200O1 K1 LCDR1
RASQDINIYLN

SEQ ID NO: 29 - protein, 7 aa, synthetic construct
  REGION 1..7: note = 200O1, h200O1 K1, h200O1 K2, h200O1 K3 LCDR2
YTSRLHS

SEQ ID NO: 30 - protein, 9 aa, synthetic construct
  REGION 1..9: note = 200O1, h200O1 K1, h200O1 K2, h200O1 K3, h200O1 K4 LCDR3
QQGHTLPYT

SEQ ID NO: 31 - protein, 126 aa, synthetic construct
  REGION 1..126: note = 175P19 VH
EVMLVESGRDLVKPGGSLRLSCAASGFTFSTYAMSWIRQTPEKRLEWVATITSAGTYTYYPDSVKGRFTISRDNAKNTLYLQMRSLRSEDTAMYYCVRHELITTVVSTDYFSMDYWGQGTSVTVSS

SEQ ID NO: 32 - DNA, 378 bp, synthetic construct
  misc_feature 1..378: note = Nucleotide sequence of 175P19 VH
  source 1..378: mol_type = other DNA
gaagtgatgctggtggagtctgggagagacttagtgaagcctggaggatccctgagactctcctgtgcagcctctggattcactttcagtacctatgccatgtcttggattcgccagactccggagaagaggctggagtgggtcgcaaccattactagtgctggtacttacacctactatccagacagtgtgaaggggcgattcaccatctccagagacaatgccaagaacaccctgtacctgcaaatgcgcagtctgaggtctgaggacacggccatgtattactgtgtaagacatgaacttattactacggtagtatctacggattacttttctatggactactggggtcaaggaacctcagtcaccgtctcctca

SEQ ID NO: 33 - protein, 5 aa, synthetic construct
  REGION 1..5: note = 175P19 HCDR1
TYAMS

SEQ ID NO: 34 - protein, 17 aa, synthetic construct
  REGION 1..17: note = 175P19 HCDR2
TITSAGTYTYYPDSVKG

SEQ ID NO: 35 - protein, 17 aa, synthetic construct
  REGION 1..17: note = 175P19 HCDR3
HELITTVVSTDYFSMDY

SEQ ID NO: 36 - protein, 111 aa, synthetic construct
  REGION 1..111: note = 175P19 VL
DIVLTQSPASLAVSLGQRATISCRASESVEYYGTSLMQWYQQKPGQPPKLLIYAASNVESGVPARFSGSGSGTDFSLNIHPVEEDDVAMYFCQQSRKVPLTFGAGTKLELK

SEQ ID NO: 37 - DNA, 333 bp, synthetic construct
  misc_feature 1..333: note = Nucleotide sequence of 175P19 VL
  source 1..333: mol_type = other DNA
gacattgtgctcacccaatctccagcttctttggctgtgtctctagggcagagagccaccatctcctgtagagccagtgaaagtgttgaatattatggcacaagtttaatgcagtggtaccaacagaaaccaggacagccacccaaactcctcatctatgctgcatccaacgtagaatctggggtccctgccaggtttagtggcagtgggtctgggacagacttcagcctcaacatccatcctgtggaggaggatgatgttgcaatgtatttctgtcagcaaagtaggaaggttccgctcacgttcggtgctgggaccaagctggagctgaaa

SEQ ID NO: 38 - protein, 15 aa, synthetic construct
  REGION 1..15: note = 175P19 LCDR1
RASESVEYYGTSLMQ

SEQ ID NO: 39 - protein, 122 aa, synthetic construct
  REGION 1..122: note = 178D4 VH
QVQLQQSGAELVKPGASVKLSCKASGYTFTSYDLNWVRQRPEQGLEWIGWTFPGDGRTKYNEKFKGKATLTTDKSSSTAYMHLSRLTSEDSAVYFCVRWDYYGRSTGYFDVWGAGTTVTVSS

SEQ ID NO: 40 - DNA, 366 bp, synthetic construct
  misc_feature 1..366: note = Nucleotide sequence of 178D4 VH
  source 1..366: mol_type = other DNA
caggttcagctgcagcagtctggagctgaactggtaaagcctggggcttcagtgaagttgtcctgcaaggcttctggctacaccttcacaagctatgatctaaactgggtgaggcagaggcctgaacagggacttgagtggattggatggacttttcctggagatggtcgtactaagtataatgagaagttcaagggcaaggccacactgactacagacaaatcctccagcacagcctacatgcacctcagcaggctgacatctgaggactctgctgtctatttctgtgtaagatgggattactacggcagaagtactgggtacttcgatgtctggggcgcagggaccacggtcaccgtctcctca

SEQ ID NO: 41 - protein, 5 aa, synthetic construct
  REGION 1..5: note = 178D4 HCDR1
SYDLN

SEQ ID NO: 42 - protein, 17 aa, synthetic construct
  REGION 1..17: note = 178D4 HCDR2
WTFPGDGRTKYNEKFKG

SEQ ID NO: 43 - protein, 13 aa, synthetic construct
  REGION 1..13: note = 178D4 HCDR3
WDYYGRSTGYFDV

SEQ ID NO: 44 - protein, 108 aa, synthetic construct
  REGION 1..108: note = 178D4 VL
QIVLTQSPAIMSASLGERVTMTCTASSSVSSSYLHWYQQRPGSSPKLWIYGTSNLASGVPARFSGSGSGTSYSLTISSMEAEDAATYYCHQYHRSPLTFGAGTKLELK

SEQ ID NO: 45 - DNA, 324 bp, synthetic construct
  misc_feature 1..324: note = Nucleotide sequence of 178D4 VL
  source 1..324: mol_type = other DNA
caaattgttctcacccagtctccagcaatcatgtctgcatctctcggggaacgggtcaccatgacctgcactgccagctcaagtgtaagttccagttacttgcactggtaccagcagaggccaggatcctcccccaaactctggatttatggcacatccaacctggcttctggagtcccagctcgcttcagtggcagtgggtctgggacctcttactctctcacaatcagcagcatggaggctgaagatgctgccacttattactgccaccagtatcatcgttccccgctcacgttcggtgctgggaccaagctggagctgaaa

SEQ ID NO: 46 - protein, 12 aa, synthetic construct
  REGION 1..12: note = 178D4 LCDR1
TASSSVSSSYLH

SEQ ID NO: 47 - protein, 7 aa, synthetic construct
  REGION 1..7: note = 178D4 LCDR2
GTSNLAS

SEQ ID NO: 48 - protein, 9 aa, synthetic construct
  REGION 1..9: note = 178D4 LCDR3
HQYHRSPLT

SEQ ID NO: 49 - protein, 126 aa, synthetic construct
  REGION 1..126: note = 185O18 VH
EVMLVESGRDLVKPGGSLKLSCAASGFTFSTYAMSWIRQTPEKRLEWVATITNYGTYTYYPDSVKGRFTISRDNAKNTLYLQMRSLRSEDTAMYYCVRHELITTVVSTDYFSMDYWGQGTSVTVSS

SEQ ID NO: 50 - DNA, 378 bp, synthetic construct
  misc_feature 1..378: note = Nucleotide sequence of 185O18 VH
  source 1..378: mol_type = other DNA
gaggtgatgctggtggagtctgggagagacttagtgaagcctggaggatccctgaaactctcctgtgcagcctctggattcactttcagtacctatgccatgtcttggattcgccagactccggagaagaggctggagtgggtcgcaaccattactaattatggtacttacacctactatccagacagtgtgaaggggcgattcaccatctccagagacaatgccaagaacaccctgtacctgcaaatgcgcagtctgaggtctgaggacacggccatgtattactgtgtaagacatgaacttattactacggtagtatctacggattacttttctatggactactggggtcaaggaacctcagtcaccgtctcctca

SEQ ID NO: 51 - protein, 5 aa, synthetic construct
  REGION 1..5: note = 185O18 HCDR1
TYAMS

SEQ ID NO: 52 - protein, 17 aa, synthetic construct
  REGION 1..17: note = 185O18 HCDR2
TITNYGTYTYYPDSVKG

SEQ ID NO: 53 - protein, 17 aa, synthetic construct
  REGION 1..17: note = 185O18 HCDR3
HELITTVVSTDYFSMDY

SEQ ID NO: 54 - protein, 111 aa, synthetic construct
  REGION 1..111: note = 185O18 VL
DIVLTQSPASLAVSLGQRATISCRASESVEDYGTSLMQWYQQKPGQPPKLLIYAASNVESGVPARFSGSGSGTDFSLNIHPVEEDDVAMYFCQQSRKVPLTFGAGTKLELK

SEQ ID NO: 55 - DNA, 333 bp, synthetic construct
  misc_feature 1..333: note = Nucleotide sequence of 185O18 VL
  source 1..333: mol_type = other DNA
gacattgtgctcacccaatctccagcttctttggctgtgtctctagggcagagagccaccatctcctgtagagccagtgaaagtgttgaagattatggcacaagtttaatgcagtggtaccaacagaaaccaggacagccacccaaactcctcatctatgctgcatccaacgtagaatctggggtccctgccaggtttagtggcagtgggtctgggacagacttcagcctcaacatccatcctgtggaggaggatgatgttgcaatgtatttctgtcagcaaagtaggaaggttccgctcacgttcggtgctgggaccaagctggagctgaaa

SEQ ID NO: 56 - protein, 15 aa, synthetic construct
  REGION 1..15: note = 185O18 LCDR1
RASESVEDYGTSLMQ

SEQ ID NO: 57 - protein, 124 aa, synthetic construct
  REGION 1..124: note = 193D22 VH
EVKLVESGGGLVKPGGSLKLSCAASGFAFSSYDMSWVRQTPEKRLEWVATISNGGSYTYYPDSVKGRFSISRDNARNTLYLQMSSLRSEDTALYYCARHPLYYGNYGWWYFDVWGAGTTVTVSS

SEQ ID NO: 58 - DNA, 372 bp, synthetic construct
  misc_feature 1..372: note = Nucleotide sequence of 193D22 VH
  source 1..372: mol_type = other DNA
gaagtgaagctggtggagtctgggggaggcttagtgaagcctggagggtccctgaaactctcctgtgcagcctctggattcgctttcagtagttatgacatgtcttgggttcgccagactccggagaagaggctggagtgggtcgcaaccattagtaatggtggtagttacacctactatccagacagtgtgaagggccgattctccatctccagagacaatgccaggaacaccctgtacctgcaaatgagcagtctgaggtctgaggacacggccttgtattactgtgcaagacatcccctctattatggtaactacggctggtggtacttcgatgtctggggcgcagggaccacggtcaccgtctcctca

SEQ ID NO: 59 - protein, 5 aa, synthetic construct
  REGION 1..5: note = 193D22, 193M7 HCDR1
SYDMS

SEQ ID NO: 60 - protein, 17 aa, synthetic construct
  REGION 1..17: note = 193D22 HCDR2
TISNGGSYTYYPDSVKG

SEQ ID NO: 61 - protein, 15 aa, synthetic construct
  REGION 1..15: note = 193D22 HCDR3
HPLYYGNYGWWYFDV

SEQ ID NO: 62 - protein, 112 aa, synthetic construct
  REGION 1..112: note = 193D22 VL
DVVMTQTPLSLPVSLGDQASISCRSSQSLVYSNGNTYLYWYLQKPGQSPKLLIYKVSNRFSGVPDRFSGSGSGTDFTLKISRVEAEDLGVYFCSQSTHVPLTFGAGTKLELK

SEQ ID NO: 63 - DNA, 336 bp, synthetic construct
  misc_feature 1..336: note = Nucleotide sequence of 193D22 VL
  source 1..336: mol_type = other DNA
gatgttgtgatgacccaaactccactctccctgcctgtcagtcttggagatcaagcctccatctcttgcagatctagtcagagccttgtatacagtaatggaaacacctatttatattggtacctgcagaagccaggccagtctccaaagctcctgatctacaaagtttccaaccgattttctggggtcccagacaggttcagtggcagtggatcagggacagatttcacactcaagatcagcagagtggaggctgaggatctgggagtttatttctgctctcaaagtacacatgttcctctcacgttcggtgctgggaccaagctggagctgaaa

SEQ ID NO: 64 - protein, 16 aa, synthetic construct
  REGION 1..16: note = 193D22 LCDR1
RSSQSLVYSNGNTYLY

SEQ ID NO: 65 - protein, 7 aa, synthetic construct
  REGION 1..7: note = 193D22, 7C8, 193M7, h7C8 K1, h7C8 K2 LCDR2
KVSNRFS

SEQ ID NO: 66 - protein, 9 aa, synthetic construct
  REGION 1..9: note = 193D22, 193M7 LCDR3
SQSTHVPLT

SEQ ID NO: 67 - protein, 126 aa, synthetic construct
  REGION 1..126: note = 151N5 VH
EVQLVESGGGLVKPGGSLKLSCAASGFTFSDFYMYWVRQTPEKRLEWVATISDGGRYTYYPDRLKGRFTISRNIAKNNLYLQMSSLKSEDTAMYYCARGRSTMITTTRNYFALDYWGQGTSVTVSS

SEQ ID NO: 68 - DNA, 378 bp, synthetic construct
  misc_feature 1..378: note = Nucleotide sequence of 151N5 VH
  source 1..378: mol_type = other DNA
gaagtgcaactggtggagtctgggggaggcttagtgaagcctggagggtccctgaaactctcctgtgctgcctctggattcactttcagtgacttttacatgtattgggttcgccagactccggaaaagaggctggagtgggtcgcaaccattagtgatggtggtcgttacacctactatccagacaggctgaaggggcgattcaccatctccagaaacattgccaagaacaacctttacctgcaaatgagcagtctgaagtctgaggacacagccatgtattactgtgcaagagggagatctactatgattacgacgacgcggaattactttgctttggactactggggtcaaggaacctcagtcaccgtctcctca

SEQ ID NO: 69 - protein, 5 aa, synthetic construct
  REGION 1..5: note = 151N5, h151N5 H1 HCDR1
DFYMY

SEQ ID NO: 70 - protein, 17 aa, synthetic construct
  REGION 1..17: note = 151N5, h151N5 H1 HCDR2
TISDGGRYTYYPDRLKG

SEQ ID NO: 71 - protein, 17 aa, synthetic construct
  REGION 1..17: note = 151N5, h151N5 H1, h151N5 H2, h151N5 H3 HCDR3
GRSTMITTTRNYFALDY

SEQ ID NO: 72 - protein, 107 aa, synthetic construct
  REGION 1..107: note = 151N5 VL
DIQMTQSSSSFSVSLGDRVTITCKASEDIYNRLAWYQQKPGDAPRLLISGAIRLETGVPSRFSGSGSGKDYTLSITSLQTEDGATYYCQQYWRTPLTFGAGIKLELK

SEQ ID NO: 73 - DNA, 321 bp, synthetic construct
  misc_feature 1..321: note = Nucleotide sequence of 151N5 VL
  source 1..321: mol_type = other DNA
gacatccagatgacacaatcttcatcctccttttctgtatctctaggagacagagtcaccattacttgcaaggcaagtgaggacatatataatcggttagcctggtatcagcagaaaccaggagatgctcctagactcttgatatctggtgctatccgtttggaaactggggttccttcaagattcagtggcagtggatctggaaaggattacactctcagcattaccagtcttcagactgaagatggtgctacttattactgtcaacagtattggagaactccgctcacgttcggtgctgggatcaagctggagctgaaa

SEQ ID NO: 74 - protein, 11 aa, synthetic construct
  REGION 1..11: note = 151N5, 174J17, h151N5 K1, h151N5 K2, h151N5 K3, h151N5 K7, h151N5K8, h151N5 K9 LCDR1
KASEDIYNRLA

SEQ ID NO: 75 - protein, 7 aa, synthetic construct
  REGION 1..7: note = 151N5 LCDR2
GAIRLET

SEQ ID NO: 76 - protein, 9 aa, synthetic construct
  REGION 1..9: note = 151N5, 174J17, h151N5 K1, h151N5 K2, h151N5 K3, h151N5 K4, h151N5K5, h151N5 K7, h151N5 K8, h151N5 K9 LCDR3
QQYWRTPLT

SEQ ID NO: 77 - protein, 122 aa, synthetic construct
  REGION 1..122: note = 156N21 VH
EVKLVESGGGLVQPGGSRKLSCAASGFTFRDYGMAWVRQAPGKGPEWVAFISNLAYSIYYADTVTGRFTISRENAKNTLYLEMSSLRSEDTAMYYCARGIHYSGRYYAMDYWGQGTSVTVSS

SEQ ID NO: 78 - DNA, 366 bp, synthetic construct
  misc_feature 1..366: note = Nucleotide sequence of 156N21 VH
  source 1..366: mol_type = other DNA
gaggtgaagctggtggagtctgggggaggcttagtgcagcctggagggtcccggaaactctcctgtgcagcctctggattcactttccgtgactacggaatggcgtgggttcgacaggctccagggaaggggcctgagtgggtagcattcattagtaatttggcatatagtatctattatgcagacactgtgacgggccgattcaccatctctagagagaatgccaagaacaccctgtacctggaaatgagcagtctgaggtctgaggacacagccatgtactactgtgcaagagggattcattactccggccgttactatgctatggactactggggtcaaggaacctcagtcaccgtctcctca

SEQ ID NO: 79 - protein, 13 aa, synthetic construct
  REGION 1..13: note = 156N21 HCDR3
GIHYSGRYYAMDY

SEQ ID NO: 80 - protein, 111 aa, synthetic construct
  REGION 1..111: note = 156N21 VL
DIVLTQSPASLAVSLGQRATISCRASKSVSTSGYSYMHWYQQKPGQPPKLLIYFASNLESGVPARFSGSGSGTDFTLNIHPVEEEDAATYYCQHSRELPPTFGGGTKLEIK

SEQ ID NO: 81 - DNA, 333 bp, synthetic construct
  misc_feature 1..333: note = Nucleotide sequence of 156N21 VL
  source 1..333: mol_type = other DNA
gacattgtgctgacacagtctcctgcttccttagctgtatctctggggcagagggccaccatctcatgtagggccagcaaaagtgtcagtacatctggctatagttatatgcactggtaccaacagaaaccaggacagccacccaaactcctcatctattttgcatccaacctagaatctggggtccctgccaggttcagtggcagtgggtctgggacagacttcaccctcaacatccatcctgtggaggaggaggatgctgcaacctattactgtcagcacagtagggagcttcctcccacgttcggaggggggaccaagctggaaataaaa

SEQ ID NO: 82 - protein, 15 aa, synthetic construct
  REGION 1..15: note = 156N21 LCDR1
RASKSVSTSGYSYMH

SEQ ID NO: 83 - protein, 7 aa, synthetic construct
  REGION 1..7: note = 156N21 LCDR2
FASNLES

SEQ ID NO: 84 - protein, 9 aa, synthetic construct
  REGION 1..9: note = 156N21 LCDR3
QHSRELPPT

SEQ ID NO: 85 - protein, 115 aa, synthetic construct
  REGION 1..115: note = 171P1 VH
QVQLEQPGAVSVRPGASVKLSCKASGYTFTSYWINWVKQRPGQGLEWIGNIYPSDSYTHYNQKFKDKATLTVDKSSTTAYMQISSPTSEDSAVYYCTREGTVVYWGQGTLLTVSA

SEQ ID NO: 86 - DNA, 346 bp, synthetic construct
  misc_feature 1..346: note = Nucleotide sequence of 171P1 VH
  source 1..346: mol_type = other DNA
caggtccaactggagcagcctggggctgtttcggtgaggcctggggcttcagtgaagctgtcctgcaaggcttctggctacaccttcaccagctactggataaactgggtgaagcagaggcctggacaaggccttgagtggatcggaaatatttatccttctgatagttatactcactacaatcaaaagttcaaggacaaggccacattgactgtagacaaatcctccaccacggcctacatgcagatcagcagcccgacatctgaggactctgcggtctattactgtacaagagaggggacggttgtttactggggccaagggactctgctcactgtctctgcag

SEQ ID NO: 87 - protein, 5 aa, synthetic construct
  REGION 1..5: note = 171P1 HCDR1
SYWIN

SEQ ID NO: 88 - protein, 17 aa, synthetic construct
  REGION 1..17: note = 171P1 HCDR2
NIYPSDSYTHYNQKFKD

SEQ ID NO: 89 - protein, 6 aa, synthetic construct
  REGION 1..6: note = 171P1 HCDR3
EGTVVY

SEQ ID NO: 90 - protein, 112 aa, synthetic construct
  REGION 1..112: note = 171P1 VL
DVVLTQTPLTLSVTIGQPASMSCKSSQSLLYSNGKTYLNWLFQRPGQSPKRLIYVVSKLDSGVPDRFTGSGSGTDFTLKISRVEAEDLGVYYCVQGTHFPFTFGSGTKLEIK

SEQ ID NO: 91 - DNA, 336 bp, synthetic construct
  misc_feature 1..336: note = Nucleotide sequence of 171P1 VL
  source 1..336: mol_type = other DNA
gatgttgtgctgacccagactccactcactttgtcggttaccattggacaaccagcctctatgtcttgcaagtcaagtcagagcctcttgtatagtaatggaaaaacctatttgaattggttattccagaggccaggccagtccccaaagcgcctaatctatgtggtgtctaaactggactctggagtccctgacaggttcactggcagtggatcaggaacagattttacactgaaaatcagcagagtggaggctgaggatttgggagtttattactgcgtgcaaggtacacattttccattcacgttcggctcggggacaaagttggaaataaaa

SEQ ID NO: 92 - protein, 16 aa, synthetic construct
  REGION 1..16: note = 171P1 LCDR1
KSSQSLLYSNGKTYLN

SEQ ID NO: 93 - protein, 7 aa, synthetic construct
  REGION 1..7: note = 171P1 LCDR2
VVSKLDS

SEQ ID NO: 94 - protein, 9 aa, synthetic construct
  REGION 1..9: note = 171P1 LCDR3
VQGTHFPFT

SEQ ID NO: 95 - protein, 118 aa, synthetic construct
  REGION 1..118: note = 6B5 VH
EVQLQQSGAELVKPGASVKLSCKASGYTFTTYWMHWVKQRPGQGLEWIGEIDPSDSYTNYNQKFKGKATLTVDKSSSTAYMQLSSLTSEDSAVYYCARSFHGNFFVYWGQGTLVTVSA

SEQ ID NO: 96 - DNA, 354 bp, synthetic construct
  misc_feature 1..354: note = Nucleotide sequence of 6B5 VH
  source 1..354: mol_type = other DNA
gaggtccaactgcagcagtctggggctgagcttgtgaagcctggggcttcagtgaagctgtcctgcaaggcttctggctacaccttcaccacctactggatgcactgggtgaagcagaggcctggacaaggccttgagtggatcggagagattgatccttctgatagttatactaactacaatcaaaagttcaagggcaaggccacgttgactgtagacaaatcctccagcacagcctacatgcagctcagcagcctgacatctgaggactctgcggtctattactgtgcaagatcgtttcatggtaacttttttgtttactggggccaagggactctggtcactgtctctgca

SEQ ID NO: 97 - protein, 5 aa, synthetic construct
  REGION 1..5: note = 6B5, h6B5 H1, h6B5 H2 HCDR1
TYWMH

SEQ ID NO: 98 - protein, 17 aa, synthetic construct
  REGION 1..17: note = 6B5, 11G10, h6B5 H1, h6B5 H2, h6B5 H3, h6B5 H4, h6B5 H5 HCDR2
EIDPSDSYTNYNQKFKG

SEQ ID NO: 99 - protein, 9 aa, synthetic construct
  REGION 1..9: note = 6B5, 6C9, h6B5 H1 HCDR3
SFHGNFFVY

SEQ ID NO: 100 - protein, 106 aa, synthetic construct
  REGION 1..106: note = 6B5 VL
QIVLTQSPAIMSASPGEKVTITCSASSSVSYMHWFQQKPGTSPKLWIYSTSNLASGVPARFSGSGSGTSYSLTISRMEAEDAATYYCQQRSSYPLTFGAGTKLELK

SEQ ID NO: 101 - DNA, 318 bp, synthetic construct
  misc_feature 1..318: note = Nucleotide sequence of 6B5 VL
  source 1..318: mol_type = other DNA
caaattgttctcacccagtctccagcaatcatgtctgcatctccaggggagaaggtcaccataacctgcagtgccagctcaagtgtaagttacatgcactggttccagcagaagccaggcacttctcccaaactctggatttatagcacatccaacctggcttctggagtccctgctcgcttcagtggcagtggatctgggacctcttactctctcacaatcagccgaatggaggctgaagatgctgccacttattactgccagcaaaggagtagttacccgctcacgttcggtgctgggaccaagctggagctgaaa

SEQ ID NO: 102 - protein, 10 aa, synthetic construct
  REGION 1..10: note = 6B5, 6C9, 11G10 LCDR1
SASSSVSYMH

SEQ ID NO: 103 - protein, 7 aa, synthetic construct
  REGION 1..7: note = 6B5, 6C9, h6B5 K1, h6B5 K4, h6B5 K5 LCDR2
STSNLAS

SEQ ID NO: 104 - protein, 9 aa, synthetic construct
  REGION 1..9: note = 6B5, 11G10, h6B5 K1, h6B5 K2, h6B5 K3, h6B5 K4, h6B5 K5, h6B5 K6LCDR3
QQRSSYPLT

SEQ ID NO: 105 - protein, 118 aa, synthetic construct
  REGION 1..118: note = 6C9 VH
QVQLQQSGAELVKPGASVKLSCKASGYTFTNYYVHWVKQRPGQGLEWIGEIDPSDSYSNYNQKFKGKATLTVDKSSSTAYMQLSSLTSEDSAVYYCARSFHGNFFVYWGQGTLVTVSA

SEQ ID NO: 106 - DNA, 354 bp, synthetic construct
  misc_feature 1..354: note = Nucleotide sequence of 6C9 VH
  source 1..354: mol_type = other DNA
caggtgcagctgcagcagtctggggctgaactggtgaagcctggggcttcggtgaagttatcctgcaaggcttctggctacaccttcaccaactactatgtgcactgggtgaagcagaggcctggacaaggccttgagtggatcggagagattgatccttctgatagttatagtaactacaatcaaaagttcaagggcaaggccacattgactgtagacaaatcctccagcacagcctacatgcagctcagcagcctgacatctgaggactctgcggtctattactgtgcaagatcgtttcatggtaacttttttgtttactggggccaagggactctggtcactgtctctgca

SEQ ID NO: 107 - protein, 5 aa, synthetic construct
  REGION 1..5: note = 6C9 HCDR1
NYYVH

SEQ ID NO: 108 - protein, 17 aa, synthetic construct
  REGION 1..17: note = 6C9 HCDR2
EIDPSDSYSNYNQKFKG

SEQ ID NO: 109 - protein, 106 aa, synthetic construct
  REGION 1..106: note = 6C9 VL
QIVLTQSPAIMSASLGEEITLTCSASSSVSYMHWFQQKPGTSPKLWIYSTSNLASGVPARFSGSGSGTSYSLTISRMEAEDAATYYCQQRSSYPPTFGGGTKLEIK

SEQ ID NO: 110 - DNA, 318 bp, synthetic construct
  misc_feature 1..318: note = Nucleotide sequence of 6C9 VL
  source 1..318: mol_type = other DNA
caaattgttctcacccagtctccagcaatcatgtctgcatctctaggggaggagatcaccctaacctgcagtgccagctcgagtgtaagttacatgcactggttccagcagaagccaggcacttctcccaaactctggatttatagcacatccaacctggcttctggagtccctgctcgcttcagtggcagtggatctgggacctcttactctctcacaatcagccgaatggaggctgaagatgctgccacttattactgccagcaaaggagtagttacccaccgacgttcggtggaggcaccaagctggaaatcaaa

SEQ ID NO: 111 - protein, 9 aa, synthetic construct
  REGION 1..9: note = 6C9 LCDR3
QQRSSYPPT

SEQ ID NO: 112 - protein, 118 aa, synthetic construct
  REGION 1..118: note = 11G10 VH
EVQLQQSGAEIVKPGASVKLSCKASGYTFTSYWMHWVKQRPGQGLEWIGEIDPSDSYTNYNQKFKGKATLTVDKSSSTAYMQLRSLTSEDSAVYYCARSFHGNLFVYWGQGTLVTVSA

SEQ ID NO: 113 - DNA, 354 bp, synthetic construct
  misc_feature 1..354: note = Nucleotide sequence of 11G10 VH
  source 1..354: mol_type = other DNA
gaggttcaactgcagcagtctggggctgagattgtgaagcctggggcttcagtgaagctgtcctgcaaggcttctggctacaccttcaccagctactggatgcactgggtgaagcagaggcctggacaaggccttgagtggatcggagagattgatccttctgatagttatactaactacaatcaaaagttcaagggcaaggccacattgactgtagacaaatcctccagcacagcctacatgcagctcagaagcctgacatctgaggactctgcggtctattactgtgcaagatcgtttcatggtaacctttttgtttactggggccaagggactctggtcactgtctctgca

SEQ ID NO: 114 - protein, 5 aa, synthetic construct
  REGION 1..5: note = 11G10 HCDR1
SYWMH

SEQ ID NO: 115 - protein, 9 aa, synthetic construct
  REGION 1..9: note = 11G10 HCDR3
SFHGNLFVY

SEQ ID NO: 116 - protein, 106 aa, synthetic construct
  REGION 1..106: note = 11G10 VL
QIVLTQSPAIMSASPGEKVTITCSASSSVSYMHWFQQKPGTSPKLWIYSTSNLATGVPARFSGSGSGTSYSLTISRMEAEDAATYYCQQRSSYPLTFGAGTKLEIK

SEQ ID NO: 117 - DNA, 318 bp, synthetic construct
  misc_feature 1..318: note = Nucleotide sequence of 11G10 VL
  source 1..318: mol_type = other DNA
caaattgttctcacccagtctccagcaatcatgtctgcatctccaggggagaaggtcaccataacctgcagtgccagctcaagtgtaagttacatgcactggttccagcagaagccaggcacttctcccaaactctggatttatagcacatccaacctggccactggagtccctgctcgcttcagtggcagtggatctgggacctcttactctctcacaatcagccgaatggaggctgaagatgctgccacttattactgccagcaaaggagtagttacccgctcacgttcggtgctgggaccaagctggaaatcaaa

SEQ ID NO: 118 - protein, 7 aa, synthetic construct
  REGION 1..7: note = 11G10 LCDR2
STSNLAT

SEQ ID NO: 119 - protein, 117 aa, synthetic construct
  REGION 1..117: note = 7C8 VH
QVTLKESGPGILQPSQTLSLTCSFSGFSLSTSGMGVSWIRQPSGKGLEWLAHIYWDDDKRYNPSLKSRLTISKDTSRNQVFLKITSVDTADTATYYCARYGKGFAYWGQGTLVTVSA

SEQ ID NO: 120 - DNA, 351 bp, synthetic construct
  misc_feature 1..351: note = Nucleotide sequence of 7C8 VH
  source 1..351: mol_type = other DNA
caggttactctgaaagagtctggccctgggatattgcagccctcccagaccctcagtctgacttgttctttctctgggttttcactgagcacttctggtatgggtgtgagctggattcgtcagccttcaggaaagggtctggagtggctggcacacatttactgggatgatgacaagcgctataacccatccctgaagagccggctcacaatctccaaggatacctccagaaaccaggtattcctcaagatcaccagtgtggacactgcagatactgccacatactactgtgctcggtatggtaaagggtttgcttactggggccaagggactctggtcactgtctctgca

SEQ ID NO: 121 - protein, 7 aa, synthetic construct
  REGION 1..7: note = 7C8, 15E11-2, h7C8 H1, h7C8 H2, h7C8 H3, h7C8 H4, h7C8 H5, h7C8H6, h7C8 H7 HCDR1
TSGMGVS

SEQ ID NO: 122 - protein, 16 aa, synthetic construct
  REGION 1..16: note = 7C8, 15E11-2, h7C8 H1, h7C8 H2, h7C8 H3, h7C8 H4, h7C8 H5, h7C8H6, h7C8 H7 HCDR2
HIYWDDDKRYNPSLKS

SEQ ID NO: 123 - protein, 7 aa, synthetic construct
  REGION 1..7: note = 7C8, h7C8 H1, h7C8 H2, h7C8 H3, h7C8 H4, h7C8 H5, h7C8 H6, h7C8H7 HCDR3
YGKGFAY

SEQ ID NO: 124 - protein, 112 aa, synthetic construct
  REGION 1..112: note = 7C8 VL
DVLMTQTPLSLPVSLGDQASISCRSSQSIVHSNGNTYLEWYLQKPGQSPKLLIYKVSNRFSGVPDRFSGSGSGTDFTLKISRVEAEDLGVYYCFQGSHVPLTFGAGTKLELK

SEQ ID NO: 125 - DNA, 337 bp, synthetic construct
  misc_feature 1..337: note = Nucleotide sequence of 7C8 VL
  source 1..337: mol_type = other DNA
gatgttttgatgacccaaactccactctccctgcctgtcagtcttggagatcaagcctccatctcttgcagatctagtcagagcattgtacatagtaatggaaacacctatttagaatggtacctgcagaaaccaggccagtctccaaagctcctgatctacaaagtttccaaccgattttctggggtcccagacaggttcagtggcagtggatcagggacagatttcacactcaagatcagcagagtggaggctgaggatctgggagtttattactgctttcaaggttcacatgttccgctcacgttcggtgctgggaccaagctggagctgaaac

SEQ ID NO: 126 - protein, 16 aa, synthetic construct
  REGION 1..16: note = 7C8, h7C8 K1 LCDR1
RSSQSIVHSNGNTYLE

SEQ ID NO: 127 - protein, 9 aa, synthetic construct
  REGION 1..9: note = 7C8, h7C8 K1, h7C8 K2 LCDR3
FQGSHVPLT

SEQ ID NO: 128 - protein, 126 aa, synthetic construct
  REGION 1..126: note = 174J17 VH
EVQLVESGGGLVKPGGSLKLSCAASGFTLSDYYMYWVRQTPEKRLEWVATISDGGRYTYYPDSVKGRFTISRDIAKNNLYIQMSSLRSEDTAMYYCARGRSTMITTTRNYLALDYWGQGTSVTVSS

SEQ ID NO: 129 - DNA, 378 bp, synthetic construct
  misc_feature 1..378: note = Nucleotide sequence of 174J17 VH
  source 1..378: mol_type = other DNA
gaagtgcagctggtggagtctgggggaggcttagtgaagcctggagggtccctgaaactctcctgtgcagcctctggattcactctcagtgactattacatgtattgggttcgccagactccggaaaagaggctggagtgggtcgcaaccattagtgatggtggtcgttacacctactatccagatagtgtgaaggggcgattcaccatctccagagacattgccaagaacaacctgtatattcaaatgagcagtctgaggtctgaggacacagccatgtattactgtgcaagagggagatctactatgattacgacgacgcggaattaccttgctttggactactggggtcaaggaacctcagtcaccgtctcctca

SEQ ID NO: 130 - protein, 5 aa, synthetic construct
  REGION 1..5: note = 174J17 HCDR1
DYYMY

SEQ ID NO: 131 - protein, 17 aa, synthetic construct
  REGION 1..17: note = 174J17 HCDR2
TISDGGRYTYYPDSVKG

SEQ ID NO: 132 - protein, 107 aa, synthetic construct
  REGION 1..107: note = 174J17 VL
DIQMTQSSSSFSVSVGDRVTVTCKASEDIYNRLAWYQQRPGNAPRLLISGATSLETGVPSRFSGSGSGKDYILSITSLQTEDVGTYYCQQYWRTPLTFGEGTKLELK

SEQ ID NO: 133 - DNA, 321 bp, synthetic construct
  misc_feature 1..321: note = Nucleotide sequence of 174J17 VL
  source 1..321: mol_type = other DNA
gacatccagatgacacaatcttcatcctccttttctgtatctgtaggagacagagtcaccgttacttgcaaggcaagtgaggacatatataatcggttagcctggtatcagcagagaccaggaaatgctcctagactcttaatatctggtgcaaccagtttggaaactggggttccttcaagattcagtggcagtggatctggaaaggattacattctcagcattaccagtcttcagactgaagatgttggtacttattactgtcaacagtattggagaactccgctcacgttcggtgaagggaccaagctggagctgaaa

SEQ ID NO: 134 - protein, 7 aa, synthetic construct
  REGION 1..7: note = 174J17 LCDR2
GATSLET

SEQ ID NO: 135 - protein, 124 aa, synthetic construct
  REGION 1..124: note = 193M7 VH
EVKLVESGGGLVKPGGSLKLSCAASGFAFSSYDMSWVRQTPEKRLEWVATISSRGTYTYYPDSVKGRFTISRNNARNTLYLQMSSLRSEDTALYYCARHPLYYGNYGYWYFDVWGAGTTVTVSS

SEQ ID NO: 136 - DNA, 372 bp, synthetic construct
  misc_feature 1..372: note = Nucleotide sequence of 193M7 VH
  source 1..372: mol_type = other DNA
gaagtgaagctggtggagtctgggggaggcttagtgaagcctggagggtccctgaaactctcctgtgcagcctctggattcgctttcagtagctatgacatgtcttgggttcgccagactccggagaagaggctggagtgggtcgcaaccattagtagtcgtggtacttacacctactatccagacagtgtgaagggccgattcaccatctccagaaacaatgccaggaacaccctgtacctgcaaatgagcagtctgaggtctgaggacacggccttgtattactgtgcaagacatcccctctattatggtaactacggctactggtacttcgatgtctggggcgcagggaccacggtcaccgtctcctca

SEQ ID NO: 137 - protein, 17 aa, synthetic construct
  REGION 1..17: note = 193M7 HCDR2
TISSRGTYTYYPDSVKG

SEQ ID NO: 138 - protein, 15 aa, synthetic construct
  REGION 1..15: note = 193M7 HCDR3
HPLYYGNYGYWYFDV

SEQ ID NO: 139 - protein, 112 aa, synthetic construct
  REGION 1..112: note = 193M7 VL
DVVMTQTPLSLPVSLGDQASISCRSSQSLVHSDGNIYLYWYLQKPGQSPKLLIYKVSNRFSGVPDRFSGSGSGTDFTLKISRVEAEDLGVYFCSQSTHVPLTFGAGTKLELK

SEQ ID NO: 140 - DNA, 336 bp, synthetic construct
  misc_feature 1..336: note = Nucleotide sequence of 193M7 VL
  source 1..336: mol_type = other DNA
gatgttgtgatgacccaaactccactctccctgcctgtcagtcttggagatcaagcctccatttcttgcagatctagtcagagccttgtacacagtgatggaaacatctatttatattggtatctgcagaagccaggccagtctccaaagctcctgatctacaaagtttccaaccgattttctggggtcccagacaggttcagtggcagtggatcagggacagatttcacactcaagatcagcagagtggaggctgaggatctgggagtttatttctgctctcaaagtacacatgttcctctcacgttcggtgctgggaccaagctggagctgaaa

SEQ ID NO: 141 - protein, 16 aa, synthetic construct
  REGION 1..16: note = 193M7 LCDR1
RSSQSLVHSDGNIYLY

SEQ ID NO: 142 - protein, 117 aa, synthetic construct
  REGION 1..117: note = 15E11-2 VH
QVTLKESGPGILQPSQTLSLTCSFSGFSLSTSGMGVSWIRQPSGKGLEWLAHIYWDDDKRYNPSLKSRLTISKVTSRNQVFLKITSVDTADTATYYCARYDKGFPYWGQGTLVTVSA

SEQ ID NO: 143 - DNA, 351 bp, synthetic construct
  misc_feature 1..351: note = Nucleotide sequence of 15E11-2 VH
  source 1..351: mol_type = other DNA
caggttactctgaaagagtctggccctgggatattgcagccctcccagaccctcagtctgacttgttctttctctgggttttcactgagcacttctggtatgggtgtgagctggattcgtcagccttcaggaaagggtctggagtggctggcacacatttactgggatgatgacaagcgctataacccatccctgaagagccggctcacaatctccaaggttacctccagaaaccaggtattcctcaagatcaccagtgtggacactgcagatactgccacatactactgtgctcggtatgataaagggtttccttactggggccaagggactctggtcactgtctctgca

SEQ ID NO: 144 - protein, 7 aa, synthetic construct
  REGION 1..7: note = 15E11-2 HCDR3
YDKGFPY

SEQ ID NO: 145 - protein, 113 aa, synthetic construct
  REGION 1..113: note = 15E11-2 VL
DTVMTQSPSSLAMSVGQKVTMSCKSSQSLLNSSNQKNYLAWYQQKPGQSPKLLIYFASTRESGVPDRFIGSGSGTDFTLTISSVQAEDLADYFCQQHYSTPLTFGAGTKLELK

SEQ ID NO: 146 - DNA, 339 bp, synthetic construct
  misc_feature 1..339: note = Nucleotide sequence of 15E11-2 VL
  source 1..339: mol_type = other DNA
gacactgtgatgacacagtctccatcctccctggctatgtcagtaggacagaaggtcactatgagctgcaagtccagtcagagccttttaaatagtagcaatcaaaagaactatttggcctggtatcagcagaaaccaggacagtctcctaaacttctgatatactttgcatccactagggaatctggggtccctgatcgcttcataggcagtggatctgggacagatttcactcttaccatcagcagtgtgcaggctgaagacctggcagattacttctgtcagcaacattatagcacgcctctcacgttcggtgctgggaccaagctggagctgaaa

SEQ ID NO: 147 - protein, 17 aa, synthetic construct
  REGION 1..17: note = 15E11-2 LCDR1
KSSQSLLNSSNQKNYLA

SEQ ID NO: 148 - protein, 7 aa, synthetic construct
  REGION 1..7: note = 15E11-2 LCDR2
FASTRES

SEQ ID NO: 149 - protein, 9 aa, synthetic construct
  REGION 1..9: note = 15E11-2 LCDR3
QQHYSTPLT

SEQ ID NO: 150 - protein, 117 aa, synthetic construct
  REGION 1..117: note = h7C8 H1 VH
QVTLKESGPALVKPTQTLTLTCTFSGFSLSTSGMGVSWIRQPPGKALEWLAHIYWDDDKRYNPSLKSRLTITKDTSRNQVVLTMTNMDPVDTATYYCARYGKGFAYWGQGTLVTVSS

SEQ ID NO: 151 - DNA, 351 bp, synthetic construct
  misc_feature 1..351: note = Nucleotide sequence of h7C8 H1 VH
  source 1..351: mol_type = other DNA
caagtgaccctgaaagagtctggccccgctctggtcaagcccacacagacactgaccctgacctgtaccttcagcggcttcagcctgagcacatctggcatgggagtgtcctggatcagacagcctcctggcaaggctctggaatggctggctcacatctactgggacgacgacaagagatacaaccccagcctgaagtccagactgaccatcaccaaggacaccagcagaaaccaggtggtgctgaccatgacaaacatggaccctgtggacaccgccacctactactgtgccagatacggcaagggcttcgcctactggggacagggaacactggtcaccgttagctct

SEQ ID NO: 152 - protein, 117 aa, synthetic construct
  REGION 1..117: note = h7C8 H2 VH
QVTLKESGPALVKPTQTLTLTCTFSGFSLSTSGMGVSWIRQPPGKALEWLAHIYWDDDKRYNPSLKSRLTITKDTSKNQVVLTMTNMDPVDTATYYCARYGKGFAYWGQGTLVTVSS

SEQ ID NO: 153 - DNA, 351 bp, synthetic construct
  misc_feature 1..351: note = Nucleotide sequence of h7C8 H2 VH
  source 1..351: mol_type = other DNA
caagtgaccctgaaagagtctggccccgctctggtcaagcccacacagacactgaccctgacctgtaccttcagcggcttcagcctgagcacatctggcatgggagtgtcctggatcagacagcctcctggcaaggctctggaatggctggctcacatctactgggacgacgacaagagatacaaccccagcctgaagtccagactgaccatcaccaaggacaccagcaaaaaccaggtggtgctgaccatgacaaacatggaccctgtggacaccgccacctactactgtgccagatacggcaagggcttcgcctactggggacagggaacactggtcaccgttagctct

SEQ ID NO: 154 - protein, 117 aa, synthetic construct
  REGION 1..117: note = h7C8 H3 VH
QVQLQESGPGLVKPSETLSLTCTFSGFSISTSGMGVSWIRQPPGKGLEWIGHIYWDDDKRYNPSLKSRVTISKDTSKNQFSLKLSSVTAADTAVYYCARYGKGFAYWGQGTLVTVSS

SEQ ID NO: 155 - DNA, 351 bp, synthetic construct
  misc_feature 1..351: note = Nucleotide sequence of h7C8 H3 VH
  source 1..351: mol_type = other DNA
caggttcagctgcaagagtctggacctggcctggtcaagcctagcgagacactgagcctgacctgtaccttcagcggcttcagcatcagcacatctggcatgggagtgtcctggatcagacagcctcctggcaaaggcctggaatggatcggccacatctactgggacgacgacaagagatacaaccccagcctgaagtccagagtgaccatcagcaaggacaccagcaaaaaccagttctccctgaagctgagcagcgtgacagccgctgataccgccgtgtactactgtgccagatacggcaagggcttcgcctactggggacagggaacactggtcaccgttagctct

SEQ ID NO: 156 - protein, 117 aa, synthetic construct
  REGION 1..117: note = h7C8 H4 VH
QVQLQESGPGLVKPSETLSLTCTFSGFSLSTSGMGVSWIRQPPGKGLEWLAHIYWDDDKRYNPSLKSRVTISKDTSRNQVSLKLSSVTAADTAVYYCARYGKGFAYWGQGTLVTVSS

SEQ ID NO: 157 - DNA, 351 bp, synthetic construct
  misc_feature 1..351: note = Nucleotide sequence of h7C8 H4 VH
  source 1..351: mol_type = other DNA
caggttcagctgcaagagtctggacctggcctggtcaagcctagcgagacactgagcctgacctgtaccttcagcggcttcagcctgagcacatctggcatgggagtgtcctggatcagacagcctcctggcaaaggcctggaatggctcgcccacatctactgggacgacgacaagagatacaaccccagcctgaagtccagagtgaccatcagcaaggacaccagcagaaaccaggtgtccctgaagctgagcagcgtgacagccgctgataccgccgtgtactactgtgccagatacggcaagggcttcgcctactggggacagggaacactggtcaccgttagctct

SEQ ID NO: 158 - protein, 117 aa, synthetic construct
  REGION 1..117: note = h7C8 H5 VH
QVQLQESGPGLVKPSETLSLTCTFSGFSLSTSGMGVSWIRQPPGKGLEWIAHIYWDDDKRYNPSLKSRVTISKDTSKNQVSLKLSSVTAADTAVYYCARYGKGFAYWGQGTLVTVSS

SEQ ID NO: 159 - DNA, 351 bp, synthetic construct
  misc_feature 1..351: note = Nucleotide sequence of h7C8 H5 VH
  source 1..351: mol_type = other DNA
caggttcagctgcaagagtctggacctggcctggtcaagcctagcgagacactgagcctgacctgtaccttcagcggcttcagcctgagcacatctggcatgggagtgtcctggatcagacagcctcctggcaaaggcctggaatggatcgcccacatctactgggacgacgacaagagatacaaccccagcctgaagtccagagtgaccatcagcaaggacaccagcaaaaaccaggtgtccctgaagctgagcagcgtgacagccgctgataccgccgtgtactactgtgccagatacggcaagggcttcgcctactggggacagggaacactggtcaccgttagctct

SEQ ID NO: 160 - protein, 117 aa, synthetic construct
  REGION 1..117: note = h7C8 H6 VH
QVQLQESGPGLVKPSETLSLTCTFSGFSISTSGMGVSWIRQPPGKGLEWIGHIYWDDDKRYNPSLKSRVTISKDTSKNQVSLKLSSVTAADTAVYYCARYGKGFAYWGQGTLVTVSS

SEQ ID NO: 161 - DNA, 351 bp, synthetic construct
  misc_feature 1..351: note = Nucleotide sequence of h7C8 H6 VH
  source 1..351: mol_type = other DNA
caggttcagctgcaagagtctggacctggcctggtcaagcctagcgagacactgagcctgacctgtaccttcagcggcttcagcatcagcacatctggcatgggagtgtcctggatcagacagcctcctggcaaaggcctggaatggatcggccacatctactgggacgacgacaagagatacaaccccagcctgaagtccagagtgaccatcagcaaggacaccagcaaaaaccaggtgtccctgaagctgagcagcgtgacagccgctgataccgccgtgtactactgtgccagatacggcaagggcttcgcctactggggacagggaacactggtcaccgttagctct

SEQ ID NO: 162 - protein, 117 aa, synthetic construct
  REGION 1..117: note = h7C8 H7 VH
QVQLQESGPGLVKPSETLSLTCTVSGFSISTSGMGVSWIRQPPGKGLEWIGHIYWDDDKRYNPSLKSRVTISKDTSKNQVSLKLSSVTAADTAVYYCARYGKGFAYWGQGTLVTVSS

SEQ ID NO: 163 - DNA, 351 bp, synthetic construct
  misc_feature 1..351: note = Nucleotide sequence of h7C8 H7 VH
  source 1..351: mol_type = other DNA
caggttcagctgcaagagtctggacctggcctggtcaagcctagcgagacactgagcctgacctgtaccgtcagcggcttcagcatcagcacatctggcatgggagtgtcctggatcagacagcctcctggcaaaggcctggaatggatcggccacatctactgggacgacgacaagagatacaaccccagcctgaagtccagagtgaccatcagcaaggacaccagcaaaaaccaggtgtccctgaagctgagcagcgtgacagccgctgataccgccgtgtactactgtgccagatacggcaagggcttcgcctactggggacagggaacactggtcaccgttagctct

SEQ ID NO: 164 - protein, 117 aa, synthetic construct
  REGION 1..117: note = h200O1 H1 VH
QVTLKESGPVLVKPTETLTLTCTVSGFSLSRYIVHWYRQPPGKALEWLAMIWGGGRIDYNSALKSRLTISKDNSKSQVVLTMTNMDPVDTATYYCARNFGENAEAYWGQGTLVTVSS

SEQ ID NO: 165 - DNA, 351 bp, synthetic construct
  misc_feature 1..351: note = Nucleotide sequence of h200O1 H1 VH
  source 1..351: mol_type = other DNA
caagtgaccctgaaagaaagcggccctgtgctggtcaagcccaccgaaacactgaccctgacctgtaccgtgtccggcttcagcctgtctcggtacatcgtgcactggtacagacagcctccaggcaaggctctggaatggctggctatgatttggggcggaggcagaatcgactacaacagcgccctgaagtccagactgaccatcagcaaggacaacagcaagagccaggtggtgctgaccatgaccaacatggaccctgtggacaccgccacctactactgcgctagaaacttcggcgagaacgccgaggcttactggggacagggaacactggtcaccgtgtctagt

SEQ ID NO: 166 - protein, 117 aa, synthetic construct
  REGION 1..117: note = h200O1 H2 VH
QVTLKESGPVLVKPTETLTLTCTVSGFSLSRYIVHWYRQPPGKALEWLAMIWGGGRIDYNSALKSRLTISKDTSKSQVVLTMTNMDPVDTATYYCARNFGENAEAYWGQGTLVTVSS

SEQ ID NO: 167 - DNA, 351 bp, synthetic construct
  misc_feature 1..351: note = Nucleotide sequence of h200O1 H2 VH
  source 1..351: mol_type = other DNA
caagtgaccctgaaagaaagcggccctgtgctggtcaagcccaccgaaacactgaccctgacctgtaccgtgtccggcttcagcctgtctcggtacatcgtgcactggtacagacagcctccaggcaaggctctggaatggctggctatgatttggggcggaggcagaatcgactacaacagcgccctgaagtccagactgaccatcagcaaggacaccagcaagagccaggtggtgctgaccatgaccaacatggaccctgtggacaccgccacctactactgcgctagaaacttcggcgagaacgccgaggcttactggggacagggaacactggtcaccgtgtctagt

SEQ ID NO: 168 - protein, 117 aa, synthetic construct
  REGION 1..117: note = h200O1 H3 VH
QVTLKESGPVLVKPTETLTLTCTVSGFSLSRYIVHWYRQPPGKALEWLAMIFGGGRIDYNSALKSRLTISKDTSKSQVVLTMTNMDPVDTATYYCARNFGENAEAYWGQGTLVTVSS

SEQ ID NO: 169 - DNA, 351 bp, synthetic construct
  misc_feature 1..351: note = Nucleotide sequence of h200O1 H3 VH
  source 1..351: mol_type = other DNA
caagtgaccctgaaagaaagcggccctgtgctggtcaagcccaccgaaacactgaccctgacctgtaccgtgtccggcttcagcctgtctcggtacatcgtgcactggtacagacagcctccaggcaaggctctggaatggctggctatgattttcggcggaggcagaatcgactacaacagcgccctgaagtccagactgaccatcagcaaggacaccagcaagagccaggtggtgctgaccatgaccaacatggaccctgtggacaccgccacctactactgcgctagaaacttcggcgagaacgccgaggcttactggggacagggaacactggtcaccgtgtctagt

SEQ ID NO: 170 - protein, 16 aa, synthetic construct
  REGION 1..16: note = h200O1 H3, h200O1 H7 HCDR2
MIFGGGRIDYNSALKS

SEQ ID NO: 171 - protein, 117 aa, synthetic construct
  REGION 1..117: note = h200O1 H4 VH
QVTLKESGPVLVKPTETLTLTCTVSGFSLSRYIVHWYRQPPGKALEWLAMIFGSGRIDYNSALKSRLTISKDTSKSQVVLTMTNMDPVDTATYYCARNFGENAEAYWGQGTLVTVSS

SEQ ID NO: 172 - DNA, 351 bp, synthetic construct
  misc_feature 1..351: note = Nucleotide sequence of h200O1 H4 VH
  source 1..351: mol_type = other DNA
caagtgaccctgaaagaaagcggccctgtgctggtcaagcccaccgaaacactgaccctgacctgtaccgtgtccggcttcagcctgtctcggtacatcgtgcactggtacagacagcctccaggcaaggctctggaatggctggctatgattttcggcagcggcagaatcgactacaacagcgccctgaagtccagactgaccatcagcaaggacaccagcaagagccaggtggtgctgaccatgaccaacatggaccctgtggacaccgccacctactactgcgctagaaacttcggcgagaacgccgaggcttactggggacagggaacactggtcaccgtgtctagt

SEQ ID NO: 173 - protein, 16 aa, synthetic construct
  REGION 1..16: note = h200O1 H4, h200O1 H8 HCDR2
MIFGSGRIDYNSALKS

SEQ ID NO: 174 - protein, 117 aa, synthetic construct
  REGION 1..117: note = h200O1 H5 VH
QVQLQESGPGLVKPSETLSLTCTVSGFSLSRYIVHWYRQPPGKGLEWIGMIWGGGRIDYNSALKSRVTISKDNSKSQVSLKLSSVTAADTAVYYCARNFGENAEAYWGQGTLVTVSS

SEQ ID NO: 175 - DNA, 351 bp, synthetic construct
  misc_feature 1..351: note = Nucleotide sequence of h200O1 H5 VH
  source 1..351: mol_type = other DNA
caggttcagctgcaagagtctggacctggcctggtcaagcctagcgagacactgagcctgacctgtaccgtgtctggcttcagcctgagccggtacatcgtgcactggtacagacagcctccaggcaaaggcctggaatggatcggcatgatttggggcggaggcagaatcgactacaacagcgccctgaagtccagagtgaccatcagcaaggacaacagcaagagccaggtgtccctgaagctgagcagcgtgacagccgctgataccgccgtgtactactgcgccagaaacttcggcgagaacgccgaggcttattggggccagggaacactggtcaccgtgtctagt

SEQ ID NO: 176 - protein, 117 aa, synthetic construct
  REGION 1..117: note = h200O1 H6 VH
QVQLQESGPGLVKPSETLSLTCTVSGFSLSRYIVHWYRQPPGKGLEWIGMIWGGGRIDYNSALKSRVTISKDTSKNQVSLKLSSVTAADTAVYYCARNFGENAEAYWGQGTLVTVSS

SEQ ID NO: 177 - DNA, 351 bp, synthetic construct
  misc_feature 1..351: note = Nucleotide sequence of h200O1 H6 VH
  source 1..351: mol_type = other DNA
caggttcagctgcaagagtctggacctggcctggtcaagcctagcgagacactgagcctgacctgtaccgtgtctggcttcagcctgagccggtacatcgtgcactggtacagacagcctccaggcaaaggcctggaatggatcggcatgatttggggcggaggcagaatcgactacaacagcgccctgaagtccagagtgaccatcagcaaggacaccagcaagaaccaggtgtccctgaagctgagcagcgtgacagccgctgataccgccgtgtactactgcgccagaaacttcggcgagaacgccgaggcttattggggccagggaacactggtcaccgtgtctagt

SEQ ID NO: 178 - protein, 117 aa, synthetic construct
  REGION 1..117: note = h200O1 H7 VH
QVQLQESGPGLVKPSETLSLTCTVSGFSLSRYIVHWYRQPPGKGLEWIGMIFGGGRIDYNSALKSRVTISKDTSKNQVSLKLSSVTAADTAVYYCARNFGENAEAYWGQGTLVTVSS

SEQ ID NO: 179 - DNA, 351 bp, synthetic construct
  misc_feature 1..351: note = Nucleotide sequence of h200O1 H7 VH
  source 1..351: mol_type = other DNA
caggttcagctgcaagagtctggacctggcctggtcaagcctagcgagacactgagcctgacctgtaccgtgtctggcttcagcctgagccggtacatcgtgcactggtacagacagcctccaggcaaaggcctggaatggatcggcatgattttcggcggaggcagaatcgactacaacagcgccctgaagtccagagtgaccatcagcaaggacaccagcaagaaccaggtgtccctgaagctgagcagcgtgacagccgctgataccgccgtgtactactgcgccagaaacttcggcgagaacgccgaggcttattggggccagggaacactggtcaccgtgtctagt

SEQ ID NO: 180 - protein, 117 aa, synthetic construct
  REGION 1..117: note = h200O1 H8 VH
QVQLQESGPGLVKPSETLSLTCTVSGFSLSRYIVHWYRQPPGKGLEWIGMIFGSGRIDYNSALKSRVTISKDTSKNQVSLKLSSVTAADTAVYYCARNFGENAEAYWGQGTLVTVSS

SEQ ID NO: 181 - DNA, 351 bp, synthetic construct
  misc_feature 1..351: note = Nucleotide sequence of h200O1 H8 VH
  source 1..351: mol_type = other DNA
caggttcagctgcaagagtctggacctggcctggtcaagcctagcgagacactgagcctgacctgtaccgtgtctggcttcagcctgagccggtacatcgtgcactggtacagacagcctccaggcaaaggcctggaatggatcggcatgattttcggcagcggcagaatcgactacaacagcgccctgaagtccagagtgaccatcagcaaggacaccagcaagaaccaggtgtccctgaagctgagcagcgtgacagccgctgataccgccgtgtactactgcgccagaaacttcggcgagaacgccgaggcttattggggccagggaacactggtcaccgtgtctagt

SEQ ID NO: 182 - protein, 117 aa, synthetic construct
  REGION 1..117: note = h200O1 H9 VH
QVTLKESGPVLVKPTETLTLTCTVSGFSLSRYIVHWYRQPPGKALEWLAMIWSGGRIDYNSALKSRLTISKDTSKSQVVLTMTNMDPVDTATYYCARNFGENAEAYWGQGTLVTVSS

SEQ ID NO: 183 - DNA, 351 bp, synthetic construct
  misc_feature 1..351: note = Nucleotide sequence of h200O1 H9 VH
  source 1..351: mol_type = other DNA
caagtgaccctgaaagaaagcggccctgtgctggtcaagcccaccgaaacactgaccctgacctgtaccgtgtccggcttcagcctgtctcggtacatcgtgcactggtacagacagcctccaggcaaggctctggaatggctggctatgatttggagcggaggcagaatcgactacaacagcgccctgaagtccagactgaccatcagcaaggacaccagcaagagccaggtggtgctgaccatgaccaacatggaccctgtggacaccgccacctactactgcgctagaaacttcggcgagaacgccgaggcttactggggacagggaacactggtcaccgtgtctagt

SEQ ID NO: 184 - protein, 16 aa, synthetic construct
  REGION 1..16: note = h200O1 H9 HCDR2
MIWSGGRIDYNSALKS

SEQ ID NO: 185 - protein, 118 aa, synthetic construct
  REGION 1..118: note = h6B5 H1 VH
QVQLVQSGAEVKKPGASVKVSCKASGYTFTTYWMHWVRQAPGQGLEWIGEIDPSDSYTNYNQKFKGRATLTVDKSSSTAYMELSSLRSEDTAVYYCARSFHGNFFVYWGQGTLVTVSS

SEQ ID NO: 186 - DNA, 354 bp, synthetic construct
  misc_feature 1..354: note = Nucleotide sequence of h6B5 H1 VH
  source 1..354: mol_type = other DNA
caggttcagctggttcagtctggcgccgaagtgaagaaacctggcgcctctgtgaaggtgtcctgcaaggctagcggctacacattcaccacctactggatgcactgggtccgacaggctccaggacagggacttgagtggatcggcgagatcgaccctagcgacagctacaccaactacaaccagaaattcaagggcagagcgaccctgaccgtggacaagtctagcagcaccgcctacatggaactgagcagcctgagaagcgaggacaccgccgtgtactactgcgccagaagcttccacggcaactttttcgtgtactggggccagggcaccctggtcacagtttcttct

SEQ ID NO: 187 - protein, 118 aa, synthetic construct
  REGION 1..118: note = h6B5 H2 VH
QVQLVQSGAEVKKPGASVKVSCKASGYTFTTYWMHWVRQAPGQGLEWMGEIDPSDSYTNYNQKFKGRVTLTVDKSSSTAYMELSSLRSEDTAVYYCARSFHGNLFVYWGQGTLVTVSS

SEQ ID NO: 188 - DNA, 354 bp, synthetic construct
  misc_feature 1..354: note = Nucleotide sequence of h6B5 H2 VH
  source 1..354: mol_type = other DNA
caggttcagctggttcagtctggcgccgaagtgaagaaacctggcgcctctgtgaaggtgtcctgcaaggctagcggctacacattcaccacctactggatgcactgggtccgacaggctccaggacagggacttgagtggatgggcgagatcgaccctagcgacagctacaccaactacaaccagaaattcaagggcagagtgaccctgaccgtggacaagtctagcagcaccgcctacatggaactgagcagcctgagaagcgaggacaccgccgtgtactactgcgccagatctttccacggcaacctgttcgtgtactggggccagggaacactggtcaccgttagctct

SEQ ID NO: 189 - protein, 9 aa, synthetic construct
  REGION 1..9: note = h6B5 H2, h6B5 H3, h6B5 H4, h6B5 H5 HCDR3
SFHGNLFVY

SEQ ID NO: 190 - protein, 118 aa, synthetic construct
  REGION 1..118: note = h6B5 H3 VH
QVQLVQSGAEVKKPGASVKVSCKASGYTFTSYWMHWVRQAPGQGLEWMGEIDPSDSYTNYNQKFKGRVTLTVDKSTSTAYMELSSLRSEDTAVYYCARSFHGNLFVYWGQGTLVTVSS

SEQ ID NO: 191 - DNA, 354 bp, synthetic construct
  misc_feature 1..354: note = Nucleotide sequence of h6B5 H3 VH
  source 1..354: mol_type = other DNA
caggttcagctggttcagtctggcgccgaagtgaagaaacctggcgcctctgtgaaggtgtcctgcaaggctagcggctacacattcaccagctactggatgcactgggtccgacaggctccaggacagggacttgagtggatgggcgagatcgaccctagcgacagctacaccaactacaaccagaaattcaagggcagagtgaccctgaccgtggacaagtctaccagcaccgcctacatggaactgagcagcctgagaagcgaggacaccgccgtgtactactgcgccagatctttccacggcaacctgttcgtgtactggggccagggaacactggtcaccgttagctct

SEQ ID NO: 192 - protein, 5 aa, synthetic construct
  REGION 1..5: note = h6B5 H3, h6B5 H4, h6B5 H5 HCDR1
SYWMH

SEQ ID NO: 193 - protein, 118 aa, synthetic construct
  REGION 1..118: note = h6B5 H4 VH
QVQLVQSGAEVKKPGASVKVSCKASGYTFTSYWMHWVRQAPGQGLEWMGEIDPSDSYTNYNQKFKGRVTMTVDKSTSTAYMELSSLRSEDTAVYYCARSFHGNLFVYWGQGTLVTVSS

SEQ ID NO: 194 - DNA, 354 bp, synthetic construct
  misc_feature 1..354: note = Nucleotide sequence of h6B5 H4 VH
  source 1..354: mol_type = other DNA
caggttcagctggttcagtctggcgccgaagtgaagaaacctggcgcctctgtgaaggtgtcctgcaaggctagcggctacacattcaccagctactggatgcactgggtccgacaggctccaggacagggacttgagtggatgggcgagatcgaccctagcgacagctacaccaactacaaccagaaattcaagggcagagtgaccatgaccgtggacaagtctaccagcaccgcctacatggaactgagcagcctgagaagcgaggacaccgccgtgtactactgcgccagatctttccacggcaacctgttcgtgtactggggccagggaacactggtcaccgttagctct

SEQ ID NO: 195 - protein, 118 aa, synthetic construct
  REGION 1..118: note = h6B5 H5 VH
QVQLVQSGAEVKKPGASVKVSCKASGYTFTSYWMHWVRQAPGQGLEWMGEIDPSDSYTNYNQKFKGRVTMTVDKSTSTVYMELSSLRSEDTAVYYCARSFHGNLFVYWGQGTLVTVSS

SEQ ID NO: 196 - DNA, 354 bp, synthetic construct
  misc_feature 1..354: note = Nucleotide sequence of h6B5 H5 VH
  source 1..354: mol_type = other DNA
caggttcagctggttcagtctggcgccgaagtgaagaaacctggcgcctctgtgaaggtgtcctgcaaggctagcggctacacattcaccagctactggatgcactgggtccgacaggctccaggacagggacttgagtggatgggcgagatcgaccctagcgacagctacaccaactacaaccagaaattcaagggcagagtgaccatgaccgtggacaagtctaccagcaccgtctacatggaactgagcagcctgagaagcgaggacaccgccgtgtactactgcgccagatctttccacggcaacctgttcgtgtactggggccagggaacactggtcaccgttagctct

SEQ ID NO: 197 - protein, 126 aa, synthetic construct
  REGION 1..126: note = h151N5 H1 VH
EVQLVESGGGLVKPGGSLRLSCAASGFTFSDFYMYWVRQAPGKGLEWVATISDGGRYTYYPDRLKGRFTISRDIAKNSLYLQMNSLRAEDTAVYYCARGRSTMITTTRNYFALDYWGQGTLVTVSS

SEQ ID NO: 198 - DNA, 378 bp, synthetic construct
  misc_feature 1..378: note = Nucleotide sequence of h151N5 H1 VH
  source 1..378: mol_type = other DNA
gaggtgcagctggttgaatctggcggaggactggttaagcctggcggctctctgagactgtcttgtgccgcttctggcttcaccttcagcgacttctacatgtactgggtccgacaggcccctggcaaaggactggaatgggtggccacaatcagcgacggcggcagatacacctactatcccgacagactgaagggcagattcaccatcagcagagatatcgccaagaacagcctgtacctgcagatgaactccctgagagccgaggacaccgccgtgtactattgtgccagaggcaggtccaccatgatcaccaccaccagaaactacttcgccctggactactggggccagggaacactggttaccgtgtctagt

SEQ ID NO: 199 - protein, 126 aa, synthetic construct
  REGION 1..126: note = h151N5 H2 VH
EVQLVESGGGLVKPGGSLRLSCAASGFTFSDYYMYWVRQAPGKGLEWVATISDGGRYTYYPDRVKGRFTISRDIAKNSLYLQMNSLRAEDTAVYYCARGRSTMITTTRNYFALDYWGQGTLVTVSS

SEQ ID NO: 200 - DNA, 378 bp, synthetic construct
  misc_feature 1..378: note = Nucleotide sequence of h151N5 H2 VH
  source 1..378: mol_type = other DNA
gaggtgcagctggttgaatctggcggaggactggttaagcctggcggctctctgagactgtcttgtgccgcttctggcttcaccttcagcgactactacatgtactgggtccgacaggcccctggcaaaggactggaatgggtggccacaatcagcgacggcggcagatacacctactatcccgacagagtgaagggcagattcaccatcagcagagatatcgccaagaacagcctgtacctgcagatgaactccctgagagccgaggacaccgccgtgtactattgtgccagaggcaggtccaccatgatcaccaccaccagaaactacttcgccctggactactggggccagggaacactggttaccgtgtctagt

SEQ ID NO: 201 - protein, 5 aa, synthetic construct
  REGION 1..5: note = h151N5 H2, h151N5 H3, h151N5 H4, h151N5 H5, h151N5 H6 HCDR1
DYYMY

SEQ ID NO: 202 - protein, 17 aa, synthetic construct
  REGION 1..17: note = h151N5 H2 HCDR2
TISDGGRYTYYPDRVKG

SEQ ID NO: 203 - protein, 126 aa, synthetic construct
  REGION 1..126: note = h151N5 H3 VH
EVQLVESGGGLVKPGGSLRLSCAASGFTFSDYYMYWVRQAPGKGLEWVSTISDGGRYTYYADRVKGRFTISRDIAKNSLYLQMNSLRAEDTAVYYCARGRSTMITTTRNYFALDYWGQGTLVTVSS

SEQ ID NO: 204 - DNA, 378 bp, synthetic construct
  misc_feature 1..378: note = Nucleotide sequence of h151N5 H3 VH
  source 1..378: mol_type = other DNA
gaggtgcagctggttgaatctggcggaggactggttaagcctggcggctctctgagactgtcttgtgccgcttctggcttcaccttcagcgactactacatgtactgggtccgacaggcccctggcaaaggactggaatgggtgtccacaatcagcgacggcggcagatacacctactatgccgacagagtgaagggcagattcaccatcagcagagatatcgccaagaacagcctgtacctgcagatgaactccctgagagccgaggacaccgccgtgtactattgtgccagaggcaggtccaccatgatcaccaccaccagaaactacttcgccctggactactggggccagggaacactggttaccgtgtctagt

SEQ ID NO: 205 - protein, 17 aa, synthetic construct
  REGION 1..17: note = h151N5 H3, h151N5 H4, h151N5 H5 HCDR2
TISDGGRYTYYADRVKG

SEQ ID NO: 206 - protein, 126 aa, synthetic construct
  REGION 1..126: note = h151N5 H4 VH
EVQLVESGGGLVKPGGSLRLSCAASGFTFSDYYMYWVRQAPGKGLEWVSTISDGGRYTYYADRVKGRFTISRDNAKNSLYLQMNSLRAEDTAVYYCARGRSTMITTTRNYLALDYWGQGTLVTVSS

SEQ ID NO: 207 - DNA, 378 bp, synthetic construct
  misc_feature 1..378: note = Nucleotide sequence of h151N5 H4 VH
  source 1..378: mol_type = other DNA
gaggtgcagctggttgaatctggcggaggactggttaagcctggcggctctctgagactgtcttgtgccgcttctggcttcaccttcagcgactactacatgtactgggtccgacaggcccctggcaaaggactggaatgggtgtccacaatcagcgacggcggcagatacacctactatgccgacagagtgaagggcagattcaccatcagcagagataacgccaagaacagcctgtacctgcagatgaactccctgagagccgaggacaccgccgtgtactattgtgccagaggcaggtccaccatgatcaccaccaccagaaactacctggctctggactactggggccagggaacactggtcacagtgtctagt

SEQ ID NO: 208 - protein, 126 aa, synthetic construct
  REGION 1..126: note = h151N5 H5 VH
EVQLVESGGGLVKPGGSLRLSCAASGFTFSDYYMYWVRQAPGKGLEWVSTISDGGRYTYYADRVKGRFTISRDNAKNSLYLQMNSLRAEDTAVYYCARGRSTLITTTRNYLALDYWGQGTLVTVSS

SEQ ID NO: 209 - DNA, 378 bp, synthetic construct
  misc_feature 1..378: note = Nucleotide sequence of h151N5 H5 VH
  source 1..378: mol_type = other DNA
gaggtgcagctggttgaatctggcggaggactggttaagcctggcggctctctgagactgtcttgtgccgcttctggcttcaccttcagcgactactacatgtactgggtccgacaggcccctggcaaaggactggaatgggtgtccacaatcagcgacggcggcagatacacctactatgccgacagagtgaagggcagattcaccatcagcagagataacgccaagaacagcctgtacctgcagatgaactccctgagagccgaggacaccgccgtgtactattgtgccagaggcaggtccaccctgatcaccaccaccagaaactacctggctctggactactggggccagggaacactggtcacagtgtctagt

SEQ ID NO: 210 - protein, 17 aa, synthetic construct
  REGION 1..17: note = h151N5 H5, h151N5 H6 HCDR3
GRSTLITTTRNYLALDY

SEQ ID NO: 211 - protein, 126 aa, synthetic construct
  REGION 1..126: note = h151N5 H6 VH
EVQLVESGGGLVKPGGSLRLSCAASGFTFSDYYMYWVRQAPGKGLEWVSTISESGRYTYYADRVKGRFTISRDNAKNSLYLQMNSLRAEDTAVYYCARGRSTLITTTRNYLALDYWGQGTLVTVSS

SEQ ID NO: 212 - DNA, 378 bp, synthetic construct
  misc_feature 1..378: note = Nucleotide sequence of h151N5 H6 VH
  source 1..378: mol_type = other DNA
gaggtgcagctggttgaatctggcggaggactggttaagcctggcggctctctgagactgtcttgtgccgcttctggcttcaccttcagcgactactacatgtactgggtccgacaggcccctggcaaaggactggaatgggtgtccacaatcagcgaaagcggcagatacacctactatgccgacagagtgaagggcagattcaccatcagcagagataacgccaagaacagcctgtacctgcagatgaactccctgagagccgaggacaccgccgtgtactattgtgccagaggcaggtccaccctgatcaccaccaccagaaactacctggctctggactactggggccagggaacactggtcacagtgtctagt

SEQ ID NO: 213 - protein, 17 aa, synthetic construct
  REGION 1..17: note = h151N5 H6 HCDR2
TISESGRYTYYADRVKG

SEQ ID NO: 214 - protein, 112 aa, synthetic construct
  REGION 1..112: note = h7C8 K1 VL
DVVMTQSPLSLPVTPGEPASISCRSSQSIVHSNGNTYLEWYLQKPGQSPKLLIYKVSNRFSGVPDRFSGSGSGTDFTLKISRVEAEDVGVYYCFQGSHVPLTFGQGTKLEIK

SEQ ID NO: 215 - DNA, 336 bp, synthetic construct
  misc_feature 1..336: note = Nucleotide sequence of h7C8 K1 VL
  source 1..336: mol_type = other DNA
gacgtggtcatgacacagagccctctgagcctgcctgtgacacctggcgaacctgccagcatcagctgtagaagcagccagagcatcgtgcacagcaacggcaacacctacctggaatggtatctgcagaagcccggccagtctcctaagctgctgatctacaaggtgtccaacagattcagcggcgtgcccgacagattctctggctctggatctggcaccgacttcaccctgaagatctccagagtggaagccgaggacgtgggcgtgtactactgcttccaaggctctcacgtgcccctgacatttggccagggcaccaagctggaaatcaag

SEQ ID NO: 216 - protein, 112 aa, synthetic construct
  REGION 1..112: note = h7C8 K2 VL
DIVMTQSPLSLPVTPGEPASISCRSSQSIVHSNGNTYLDWYLQKPGQSPQLLIYKVSNRFSGVPDRFSGSGSGTDFTLKISRVEAEDVGVYYCFQGSHVPLTFGQGTKLEIK

SEQ ID NO: 217 - DNA, 336 bp, synthetic construct
  misc_feature 1..336: note = Nucleotide sequence of h7C8 K2 VL
  source 1..336: mol_type = other DNA
gacatcgtcatgacacagagccctctgagcctgcctgtgacacctggcgaacctgccagcatcagctgtagaagcagccagagcatcgtgcacagcaacggcaacacctacctggactggtatctgcagaagcccggccagtctcctcagctgctgatctacaaggtgtccaacagattcagcggcgtgcccgacagattctctggctctggatctggcaccgacttcaccctgaagatctccagagtggaagccgaggacgtgggcgtgtactactgcttccaaggctctcacgtgcccctgacatttggccagggcaccaagctggaaatcaag

SEQ ID NO: 218 - protein, 16 aa, synthetic construct
  REGION 1..16: note = h7C8 K2 LCDR1
RSSQSIVHSNGNTYLD

SEQ ID NO: 219 - protein, 107 aa, synthetic construct
  REGION 1..107: note = h200O1 K1 VL
DIQMTQSPSSLSASVGDRVTITCRASQDINIYLNWYQQKPGKVVKLLIYYTSRLHSGVPSRFSGSGSGTDFTLTISSLQPEDVATYFCQQGHTLPYTFGQGTKLEIK

SEQ ID NO: 220 - DNA, 321 bp, synthetic construct
  misc_feature 1..321: note = Nucleotide sequence of h200O1 K1 VL
  source 1..321: mol_type = other DNA
gacatccagatgacacagagccctagcagcctgtctgccagcgtgggagacagagtgaccatcacctgtagagccagccaggacatcaacatctacctgaactggtatcagcagaaacccggcaaggtggtcaagctgctgatctactacaccagcagactgcacagcggcgtgccctctagattttctggcagcggctctggcaccgacttcaccctgacaatctctagcctgcagcctgaggacgtggcaacctacttctgccagcaaggccacacactgccctacacatttggccagggcaccaagctggaaatcaag

SEQ ID NO: 221 - protein, 107 aa, synthetic construct
  REGION 1..107: note = h200O1 K2 VL
DIQMTQSPSSLSASVGDRVTITCRASQDISIYLNWYQQKPGKVPKLLIYYTSRLHSGVPSRFSGSGSGTDFTLTISSLQPEDVATYFCQQGHTLPYTFGQGTKLEIK

SEQ ID NO: 222 - DNA, 321 bp, synthetic construct
  misc_feature 1..321: note = Nucleotide sequence of h200O1 K2 VL
  source 1..321: mol_type = other DNA
gacatccagatgacacagagccctagcagcctgtctgccagcgtgggagacagagtgaccatcacctgtagagccagccaggacatcagcatctacctgaactggtatcagcagaaacccggcaaggtgcccaagctgctgatctactacaccagcagactgcacagcggcgtgccctctagattttctggcagcggctctggcaccgacttcaccctgacaatctctagcctgcagcctgaggacgtggcaacctacttctgccagcaaggccacacactgccctacacatttggccagggcaccaagctggaaatcaag

SEQ ID NO: 223 - protein, 11 aa, synthetic construct
  REGION 1..11: note = h200O1 K2 LCDR1
RASQDISIYLN

SEQ ID NO: 224 - protein, 107 aa, synthetic construct
  REGION 1..107: note = h200O1 K3 VL
DIQMTQSPSSLSASVGDRVTITCRASQGISIYLNWYQQKPGKVPKLLIYYTSRLHSGVPSRFSGSGSGTDFTLTISSLQPEDVATYFCQQGHTLPYTFGQGTKLEIK

SEQ ID NO: 225 - DNA, 321 bp, synthetic construct
  misc_feature 1..321: note = Nucleotide sequence of h200O1 K3 VL
  source 1..321: mol_type = other DNA
gacatccagatgacacagagccctagcagcctgtctgccagcgtgggagacagagtgaccatcacctgtagagccagccagggcatcagcatctacctgaactggtatcagcagaaacccggcaaggtgcccaagctgctgatctactacaccagcagactgcacagcggcgtgccctctagattttctggcagcggctctggcaccgacttcaccctgacaatctctagcctgcagcctgaggacgtggcaacctacttctgccagcaaggccacacactgccctacacatttggccagggcaccaagctggaaatcaag

SEQ ID NO: 226 - protein, 11 aa, synthetic construct
  REGION 1..11: note = h200O1 K3, h200O1 K4 LCDR1
RASQGISIYLN

SEQ ID NO: 227 - protein, 107 aa, synthetic construct
  REGION 1..107: note = h200O1 K4 VL
DIQMTQSPSSLSASVGDRVTITCRASQGISIYLNWYQQKPGKVPKLLIYYASRLHSGVPSRFSGSGSGTDFTLTISSLQPEDVATYFCQQGHTLPYTFGQGTKLEIK

SEQ ID NO: 228 - DNA, 321 bp, synthetic construct
  misc_feature 1..321: note = Nucleotide sequence of h200O1 K4 VL
  source 1..321: mol_type = other DNA
gacatccagatgacacagagccctagcagcctgtctgccagcgtgggagacagagtgaccatcacctgtagagccagccagggcatcagcatctacctgaactggtatcagcagaaacccggcaaggtgcccaagctgctgatctactacgccagcagactgcacagcggcgtgccctctagattttctggcagcggctctggcaccgacttcaccctgacaatctctagcctgcagcctgaggacgtggcaacctacttctgccagcaaggccacacactgccctacacatttggccagggcaccaagctggaaatcaag

SEQ ID NO: 229 - protein, 7 aa, synthetic construct
  REGION 1..7: note = h200O1 K4 LCDR2
YASRLHS

SEQ ID NO: 230 - protein, 106 aa, synthetic construct
  REGION 1..106: note = h6B5 K1 VL
EIVLTQSPATLSLSPGERATLSCRASSSVSYMHWFQQKPGQAPRLWIYSTSNLASGIPARFSGSGSGTDYTLTISRLEPEDFAVYYCQQRSSYPLTFGQGTKLEIK

SEQ ID NO: 231 - DNA, 318 bp, synthetic construct
  misc_feature 1..318: note = Nucleotide sequence of h6B5 K1 VL
  source 1..318: mol_type = other DNA
gagatcgtgctgacacagagccctgccacactgtcactgtctccaggcgagagagccacactgagctgtagagccagcagcagcgtgtcctacatgcactggttccagcagaagcctggacaggcccctagactgtggatctacagcacaagcaacctggccagcggcatccccgctagattttctggcagcggcagcggaaccgactacaccctgacaatcagcagactggaacccgaggacttcgccgtgtactactgccagcagagaagcagctaccctctgacattcggccagggcaccaagctggaaatcaag

SEQ ID NO: 232 - protein, 10 aa, synthetic construct
  REGION 1..10: note = h6B5 K1, h6B5 K2, h6B5 K3, h6B5 K4, h6B5 K5, h6B5 K6 LCDR1
RASSSVSYMH

SEQ ID NO: 233 - protein, 106 aa, synthetic construct
  REGION 1..106: note = h6B5 K2 VL
EIVLTQSPATLSLSPGERATLSCRASSSVSYMHWFQQKPGQAPRLLIYSTSNLATGIPARFSGSGSGTDYTLTISRLEPEDFAVYYCQQRSSYPLTFGQGTKLEIK

SEQ ID NO: 234 - DNA, 318 bp, synthetic construct
  misc_feature 1..318: note = Nucleotide sequence of h6B5 K2 VL
  source 1..318: mol_type = other DNA
gagatcgtgctgacacagagccctgccacactgtcactgtctccaggcgagagagccacactgagctgtagagccagcagcagcgtgtcctacatgcactggttccagcagaagcctggacaggcccctagactgctgatctacagcacaagcaacctggccacaggcatccccgctagattttctggcagcggcagcggaaccgactacaccctgacaatcagcagactggaacccgaggacttcgccgtgtactactgccagcagagaagcagctaccctctgacattcggccagggcaccaagctggaaatcaag

SEQ ID NO: 235 - protein, 7 aa, synthetic construct
  REGION 1..7: note = h6B5 K2 LCDR2
STSNLAT

SEQ ID NO: 236 - protein, 106 aa, synthetic construct
  REGION 1..106: note = h6B5 K3 VL
EIVLTQSPATLSLSPGERATLSCRASSSVSYMHWFQQKPGQAPRLLIYSTSSRATGIPARFSGSGSGTDYTLTISRLEPEDFAVYYCQQRSSYPLTFGQGTKLEIK

SEQ ID NO: 237 - DNA, 318 bp, synthetic construct
  misc_feature 1..318: note = Nucleotide sequence of h6B5 K3 VL
  source 1..318: mol_type = other DNA
gagatcgtgctgacacagagccctgccacactgtcactgtctccaggcgagagagccacactgagctgtagagccagcagcagcgtgtcctacatgcactggttccagcagaagcctggacaggcccctagactgctgatctacagcacaagcagcagggccacaggcatccccgctagattttctggcagcggcagcggaaccgactacaccctgacaatcagcagactggaacccgaggacttcgccgtgtactactgccagcagagaagcagctaccctctgacattcggccagggcaccaagctggaaatcaag

SEQ ID NO: 238 - protein, 7 aa, synthetic construct
  REGION 1..7: note = h6B5 K3 LCDR2
STSSRAT

SEQ ID NO: 239 - protein, 106 aa, synthetic construct
  REGION 1..106: note = h6B5 K4 VL
DIQLTQSPSSLSASVGDRVTITCRASSSVSYMHWFQQKPGKAPKLWIYSTSNLASGVPSRFSGSGSGTDYTLTISSLQPEDFATYYCQQRSSYPLTFGQGTKLEIK

SEQ ID NO: 240 - DNA, 318 bp, synthetic construct
  misc_feature 1..318: note = Nucleotide sequence of h6B5 K4 VL
  source 1..318: mol_type = other DNA
gacatccagctgacacagagcccttctagcctgtctgccagcgtgggcgacagagtgaccatcacatgtagagccagcagcagcgtgtcctacatgcactggttccagcagaagcctggcaaggcccctaagctgtggatctacagcacaagcaacctggcctcaggcgtgccctctagattttctggcagcggctctggcaccgactacaccctgacaatctctagcctgcagcctgaggacttcgccacctactactgccagcagagaagcagctaccctctgacattcggccagggcaccaagctggaaatcaag

SEQ ID NO: 241 - protein, 106 aa, synthetic construct
  REGION 1..106: note = h6B5 K5 VL
DIQMTQSPSSLSASVGDRVTITCRASSSVSYMHWFQQKPGKAPKLLIYSTSNLASGVPSRFSGSGSGTDYTLTISSLQPEDFATYYCQQRSSYPLTFGQGTKLEIK

SEQ ID NO: 242 - DNA, 318 bp, synthetic construct
  misc_feature 1..318: note = Nucleotide sequence of h6B5 K5 VL
  source 1..318: mol_type = other DNA
gacatccagatgacacagagcccttctagcctgtctgccagcgtgggcgacagagtgaccatcacatgtagagccagcagcagcgtgtcctacatgcactggttccagcagaagcctggcaaggcccctaagctgctgatctacagcacaagcaacctggcctcaggcgtgccctctagattttctggcagcggctctggcaccgactacaccctgacaatctctagcctgcagcctgaggacttcgccacctactactgccagcagagaagcagctaccctctgacattcggccagggcaccaagctggaaatcaag

SEQ ID NO: 243 - protein, 106 aa, synthetic construct
  REGION 1..106: note = h6B5 K6 VL
DIQMTQSPSSLSASVGDRVTITCRASSSVSYMHWFQQKPGKAPKLLIYSTSSLQSGVPSRFSGSGSGTDYTLTISSLQPEDFATYYCQQRSSYPLTFGQGTKLEIK

SEQ ID NO: 244 - DNA, 318 bp, synthetic construct
  misc_feature 1..318: note = Nucleotide sequence of h6B5 K6 VL
  source 1..318: mol_type = other DNA
gacatccagatgacacagagcccttctagcctgtctgccagcgtgggcgacagagtgaccatcacatgtagagccagcagcagcgtgtcctacatgcactggttccagcagaagcctggcaaggcccctaagctgctgatctacagcacaagcagcctgcagtcaggcgtgccctctagattttctggcagcggctctggcaccgactacaccctgacaatctctagcctgcagcctgaggacttcgccacctactactgccagcagagaagcagctaccctctgacattcggccagggcaccaagctggaaatcaag

SEQ ID NO: 245 - protein, 7 aa, synthetic construct
  REGION 1..7: note = h6B5 K6 LCDR2
STSSLQS

SEQ ID NO: 246 - protein, 107 aa, synthetic construct
  REGION 1..107: note = h151N5 K1 VL
DIQMTQSPSSLSASVGDRVTITCKASEDIYNRLAWYQQKPGKAPKLLISGATSLETGVPSRFSGSGSGKDYTLTISSLQPEDIATYYCQQYWRTPLTFGQGTKLEIK

SEQ ID NO: 247 - DNA, 321 bp, synthetic construct
  misc_feature 1..321: note = Nucleotide sequence of h151N5 K1 VL
  source 1..321: mol_type = other DNA
gacatccagatgacacagagccctagcagcctgtctgccagcgtgggagacagagtgaccatcacctgtaaggccagcgaggacatctacaacagactggcctggtatcagcagaagcccggcaaggctcctaagctgctgatctctggcgccacctctctggaaacaggcgtgccatctagattcagcggcagcggctctggcaaggactacaccctgacaatcagcagcctgcagcctgaggatatcgccacctactactgccagcagtactggcggacccctctgacatttggccagggcaccaagctggaaatcaag

SEQ ID NO: 248 - protein, 7 aa, synthetic construct
  REGION 1..7: note = h151N5 K1, h151N5 K2 LCDR2
GATSLET

SEQ ID NO: 249 - protein, 107 aa, synthetic construct
  REGION 1..107: note = h151N5 K2 VL
DIQMTQSPSSLSASVGDRVTITCKASEDIYNRLAWYQQKPGKAPKLLISGATSLETGVPSRFSGSGSGKDYTLTISSLQPEDVATYYCQQYWRTPLTFGQGTKLEIK

SEQ ID NO: 250 - DNA, 321 bp, synthetic construct
  misc_feature 1..321: note = Nucleotide sequence of h151N5 K2 VL
  source 1..321: mol_type = other DNA
gacatccagatgacacagagccctagcagcctgtctgccagcgtgggagacagagtgaccatcacctgtaaggccagcgaggacatctacaacagactggcctggtatcagcagaagcccggcaaggctcctaagctgctgatctctggcgccacctctctggaaacaggcgtgccatctagattcagcggcagcggctctggcaaggactacaccctgacaatcagcagcctgcagcctgaggatgtcgccacctactactgccagcagtactggcggacccctctgacatttggccagggcaccaagctggaaatcaag

SEQ ID NO: 251 - protein, 107 aa, synthetic construct
  REGION 1..107: note = h151N5 K3 VL
DIQMTQSPSSLSASVGDRVTITCKASEDIYNRLAWYQQKPGKAPKLLIYGATSLQSGVPSRFSGSGSGKDYTLTISSLQPEDVATYYCQQYWRTPLTFGQGTKLEIK

SEQ ID NO: 252 - DNA, 321 bp, synthetic construct
  misc_feature 1..321: note = Nucleotide sequence of h151N5 K3 VL
  source 1..321: mol_type = other DNA
gacatccagatgacacagagccctagcagcctgtctgccagcgtgggagacagagtgaccatcacctgtaaggccagcgaggacatctacaacagactggcctggtatcagcagaagcccggcaaggctcctaagctgctgatctatggcgccacctctctgcaatcaggcgtgccatctagattcagcggcagcggctctggcaaggactacaccctgacaatcagcagcctgcagcctgaggatgtcgccacctactactgccagcagtactggcggacccctctgacatttggccagggcaccaagctggaaatcaag

SEQ ID NO: 253 - protein, 7 aa, synthetic construct
  REGION 1..7: note = h151N5 K3 LCDR2
GATSLQS

SEQ ID NO: 254 - protein, 107 aa, synthetic construct
  REGION 1..107: note = h151N5 K4 VL
DIQMTQSPSSLSASVGDRVTITCKASQDIYNRLAWYQQKPGKVPKLLIYAATSLQSGVPSRFSGSGSGKDYTLTISSLQPEDVATYYCQQYWRTPLTFGQGTKLEIK

SEQ ID NO: 255 - DNA, 321 bp, synthetic construct
  misc_feature 1..321: note = Nucleotide sequence of h151N5 K4 VL
  source 1..321: mol_type = other DNA
gacatccagatgacacagagccctagcagcctgtctgccagcgtgggagacagagtgaccatcacctgtaaggccagccaggacatctacaacagactggcctggtatcagcagaagcccggcaaggttcctaagctgctgatctatgccgccacctctctgcaatcaggcgtgccatctagattcagcggcagcggctctggcaaggactacaccctgacaatcagcagcctgcagcctgaggatgtcgccacctactactgccagcagtactggcggacccctctgacatttggccagggcaccaagctggaaatcaag

SEQ ID NO: 256 - protein, 11 aa, synthetic construct
  REGION 1..11: note = h151N5 K4 LCDR1
KASQDIYNRLA

SEQ ID NO: 257 - protein, 7 aa, synthetic construct
  REGION 1..7: note = h151N5 K4 LCDR2
AATSLQS

SEQ ID NO: 258 - protein, 107 aa, synthetic construct
  REGION 1..107: note = h151N5 K5 VL
DIQMTQSPSSLSASVGDRVTITCKASQGIYNRLAWYQQKPGKVPKLLIYAASTLQSGVPSRFSGSGSGKDYTLTISSLQPEDVATYYCQQYWRTPLTFGQGTKLEIK

SEQ ID NO: 259 - DNA, 321 bp, synthetic construct
  misc_feature 1..321: note = Nucleotide sequence of h151N5 K5 VL
  source 1..321: mol_type = other DNA
gacatccagatgacacagagccctagcagcctgtctgccagcgtgggagacagagtgaccatcacctgtaaggccagccagggcatctacaacagactggcctggtatcagcagaagcccggcaaggttcctaagctgctgatctatgccgcctccactctgcaatcaggcgtgccatctagattcagcggcagcggctctggcaaggactacaccctgacaatcagcagcctgcagcctgaggatgtcgccacctactactgccagcagtactggcggacccctctgacatttggccagggcaccaagctggaaatcaag

SEQ ID NO: 260 - protein, 11 aa, synthetic construct
  REGION 1..11: note = h151N5 K5, h151N5 K6 LCDR1
KASQGIYNRLA

SEQ ID NO: 261 - protein, 7 aa, synthetic construct
  REGION 1..7: note = h151N5 K5, h151N5 K6 LCDR2
AASTLQS

SEQ ID NO: 262 - protein, 107 aa, synthetic construct
  REGION 1..107: note = h151N5 K6 VL
DIQMTQSPSSLSASVGDRVTITCKASQGIYNRLAWYQQKPGKVPKLLIYAASTLQSGVPSRFSGSGSGKDYTLTISSLQPEDVATYYCQQYYRTPLTFGQGTKLEIK

SEQ ID NO: 263 - DNA, 321 bp, synthetic construct
  misc_feature 1..321: note = Nucleotide sequence of h151N5 K6 VL
  source 1..321: mol_type = other DNA
gacatccagatgacacagagccctagcagcctgtctgccagcgtgggagacagagtgaccatcacctgtaaggccagccagggcatctacaacagactggcctggtatcagcagaagcccggcaaggttcctaagctgctgatctatgccgcctccactctgcaatcaggcgtgccatctagattcagcggcagcggctctggcaaggactacaccctgacaatcagcagcctgcagcctgaggatgtcgccacctactactgccagcagtactaccggacccctctgacatttggccagggcaccaagctggaaatcaag

SEQ ID NO: 264 - protein, 9 aa, synthetic construct
  REGION 1..9: note = h151N5 K6 LCDR3
QQYYRTPLT

SEQ ID NO: 265 - protein, 107 aa, synthetic construct
  REGION 1..107: note = h151N5 K7 VL
DIQMTQSPSSLSASVGDRVTITCKASEDIYNRLAWYQQKPGKAPKLLISGAIRLETGVPSRFSGSGSGKDYTLTISSLQPEDIATYYCQQYWRTPLTFGQGTKLEIK

SEQ ID NO: 266 - DNA, 321 bp, synthetic construct
  misc_feature 1..321: note = Nucleotide sequence of h151N5 K7 VL
  source 1..321: mol_type = other DNA
gacatccagatgacacagagccctagcagcctgtctgccagcgtgggagacagagtgaccatcacctgtaaggccagcgaggacatctacaacagactggcctggtatcagcagaagcccggcaaggctcctaagctgctgatctctggcgccatcagactggaaacaggcgtgccatctagattcagcggcagcggctctggcaaggactacaccctgacaatcagcagcctgcagcctgaggatatcgccacctactactgccagcagtactggcggacccctctgacatttggccagggcaccaagctggaaatcaag

SEQ ID NO: 267 - protein, 107 aa, synthetic construct
  REGION 1..107: note = h151N5 K8 VL
DIQMTQSPSSLSASVGDRVTITCKASEDIYNRLAWYQQKPGKAPKLLISGAIRLETGVPSRFSGSGSGKDYTLTISSLQPEDVATYYCQQYWRTPLTFGQGTKLEIK

SEQ ID NO: 268 - DNA, 321 bp, synthetic construct
  misc_feature 1..321: note = Nucleotide sequence of h151N5 K8 VL
  source 1..321: mol_type = other DNA
gacatccagatgacacagagccctagcagcctgtctgccagcgtgggagacagagtgaccatcacctgtaaggccagcgaggacatctacaacagactggcctggtatcagcagaagcccggcaaggctcctaagctgctgatctctggcgccatcagactggaaacaggcgtgccatctagattcagcggcagcggctctggcaaggactacaccctgacaatcagcagcctgcagcctgaggatgtcgccacctactactgccagcagtactggcggacccctctgacatttggccagggcaccaagctggaaatcaag

SEQ ID NO: 269 - protein, 107 aa, synthetic construct
  REGION 1..107: note = h151N5 K9 VL
DIQMTQSPSSLSASVGDRVTITCKASEDIYNRLAWYQQKPGKAPKLLIYGAIRLETGVPSRFSGSGSGKDYTLTISSLQPEDVATYYCQQYWRTPLTFGQGTKLEIK

SEQ ID NO: 270 - DNA, 321 bp, synthetic construct
  misc_feature 1..321: note = Nucleotide sequence of h151N5 K9 VL
  source 1..321: mol_type = other DNA
gacatccagatgacacagagccctagcagcctgtctgccagcgtgggagacagagtgaccatcacctgtaaggccagcgaggacatctacaacagactggcctggtatcagcagaagcccggcaaggctcctaagctgctgatctatggcgccatcagactggaaacaggcgtgccatctagattcagcggcagcggctctggcaaggactacaccctgacaatcagcagcctgcagcctgaggatgtcgccacctactactgccagcagtactggcggacccctctgacatttggccagggcaccaagctggaaatcaag

SEQ ID NO: 271 - protein, 447 aa, synthetic construct
  REGION 1..447: note = Heavy chain of h7C8 H6K2 hIgG1 LA
QVQLQESGPGLVKPSETLSLTCTFSGFSISTSGMGVSWIRQPPGKGLEWIGHIYWDDDKRYNPSLKSRVTISKDTSKNQVSLKLSSVTAADTAVYYCARYGKGFAYWGQGTLVTVSSASTKGPSVFPLAPSSKSTSGGTAALGCLVKDYFPEPVTVSWNSGALTSGVHTFPAVLQSSGLYSLSSVVTVPSSSLGTQTYICNVNHKPSNTKVDKRVEPKSCDKTHTCPPCPAPELLGGPSVFLFPPKPKDTLMISRTPEVTCVVVDVSHEDPEVKFNWYVDGVEVHNAKTKPREEQYNSTYRVVSVLTVLHQDWLNGKEYKCKVSNKALPAPIEKTISKAKGQPREPQVYTLPPSREEMTKNQVSLTCLVKGFYPSDIAVEWESNGQPENNYKTTPPVLDSDGSFFLYSKLTVDKSRWQQGNVFSCSVLHEALHAHYTQKSLSLSPGK

SEQ ID NO: 272 - DNA, 1341 bp, synthetic construct
  misc_feature 1..1341: note = Nucleotide sequence of heavy chain of h7C8 H6K2 hIgG1 LA
  source 1..1341: mol_type = other DNA
caggttcagctgcaagagtctggacctggcctggtcaagcctagcgagacactgagcctgacctgtaccttcagcggcttcagcatcagcacatctggcatgggagtgtcctggatcagacagcctcctggcaaaggcctggaatggatcggccacatctactgggacgacgacaagagatacaaccccagcctgaagtccagagtgaccatcagcaaggacaccagcaaaaaccaggtgtccctgaagctgagcagcgtgacagccgctgataccgccgtgtactactgtgccagatacggcaagggcttcgcctactggggacagggaacactggtcaccgttagctctgctagcaccaagggcccatccgtcttccccctggcaccctcctccaagagcacctctgggggcacagcggccctgggctgcctggtcaaggactacttccccgaaccggtgacggtgtcgtggaactcaggcgccctgaccagcggcgtgcacaccttcccggctgtcctacagtcctcaggactctactccctcagcagcgtggtgaccgtgccctccagcagcttgggcacccagacctacatctgcaacgtgaatcacaagcccagcaacaccaaggtggacaagagagttgagcccaaatcttgtgacaaaactcacacatgcccaccgtgcccagcacctgaactcctggggggaccgtcagtcttcctcttccccccaaaacccaaggacaccctcatgatctcccggacccctgaggtcacatgcgtggtggtggacgtgagccacgaagaccctgaggtcaagttcaactggtacgtggacggcgtggaggtgcataatgccaagacaaagccgcgggaggagcagtacaacagcacgtaccgtgtggtcagcgtcctcaccgtcctgcaccaggactggctgaatggcaaggagtacaagtgcaaggtctccaacaaagccctcccagcccccatcgagaaaaccatctccaaagccaaagggcagccccgagaaccacaggtgtacaccctgcccccatcccgggaggagatgaccaagaaccaggtcagcctgacctgcctggtcaaaggcttctatcccagcgacatcgccgtggagtgggagagcaatgggcagccggagaacaactacaagaccacgcctcccgtgctggactccgacggctccttcttcctctatagcaagctcaccgtggacaagagcaggtggcagcaggggaacgtcttctcatgctccgtgctgcatgaggctctgcacgcccactacacgcagaagtccctctccctgtctccgggtaaa

SEQ ID NO: 273 - protein, 219 aa, synthetic construct
  REGION 1..219: note = Light chain of h7C8 H6K2 hIgG1 LA
DIVMTQSPLSLPVTPGEPASISCRSSQSIVHSNGNTYLDWYLQKPGQSPQLLIYKVSNRFSGVPDRFSGSGSGTDFTLKISRVEAEDVGVYYCFQGSHVPLTFGQGTKLEIKRTVAAPSVFIFPPSDEQLKSGTASVVCLLNNFYPREAKVQWKVDNALQSGNSQESVTEQDSKDSTYSLSSTLTLSKADYEKHKVYACEVTHQGLSSPVTKSFNRGEC

SEQ ID NO: 274 - DNA, 657 bp, synthetic construct
  misc_feature 1..657: note = Nucleotide sequence of light chain of h7C8 H6K2 hIgG1 LA
  source 1..657: mol_type = other DNA
gacatcgtcatgacacagagccctctgagcctgcctgtgacacctggcgaacctgccagcatcagctgtagaagcagccagagcatcgtgcacagcaacggcaacacctacctggactggtatctgcagaagcccggccagtctcctcagctgctgatctacaaggtgtccaacagattcagcggcgtgcccgacagattctctggctctggatctggcaccgacttcaccctgaagatctccagagtggaagccgaggacgtgggcgtgtactactgcttccaaggctctcacgtgcccctgacatttggccagggcaccaagctggaaatcaagcgaactgtggctgcaccatctgtcttcatcttcccgccatctgatgagcagttgaaatctggaactgcctctgttgtgtgcctgctgaataacttctatcccagagaggccaaagtacagtggaaggtggataacgccctccaatcgggtaactcccaggagagtgtcacagagcaggacagcaaggacagcacctacagcctcagcagcaccctgacgctgagcaaagcagactacgagaaacacaaagtctacgcctgcgaagtcacccatcagggcctgagctcgcccgtcacaaagagcttcaacaggggagagtgt

SEQ ID NO: 275 - protein, 447 aa, synthetic construct
  REGION 1..447: note = Heavy chain of h200O1 H1K1 hIgG1 LA
QVTLKESGPVLVKPTETLTLTCTVSGFSLSRYIVHWYRQPPGKALEWLAMIWGGGRIDYNSALKSRLTISKDNSKSQVVLTMTNMDPVDTATYYCARNFGENAEAYWGQGTLVTVSSASTKGPSVFPLAPSSKSTSGGTAALGCLVKDYFPEPVTVSWNSGALTSGVHTFPAVLQSSGLYSLSSVVTVPSSSLGTQTYICNVNHKPSNTKVDKRVEPKSCDKTHTCPPCPAPELLGGPSVFLFPPKPKDTLMISRTPEVTCVVVDVSHEDPEVKFNWYVDGVEVHNAKTKPREEQYNSTYRVVSVLTVLHQDWLNGKEYKCKVSNKALPAPIEKTISKAKGQPREPQVYTLPPSREEMTKNQVSLTCLVKGFYPSDIAVEWESNGQPENNYKTTPPVLDSDGSFFLYSKLTVDKSRWQQGNVFSCSVLHEALHAHYTQKSLSLSPGK

SEQ ID NO: 276 - DNA, 1341 bp, synthetic construct
  misc_feature 1..1341: note = Nucleotide sequence of heavy chain of h200O1 H1K1 hIgG1 LA
  source 1..1341: mol_type = other DNA
caagtgaccctgaaagaaagcggccctgtgctggtcaagcccaccgaaacactgaccctgacctgtaccgtgtccggcttcagcctgtctcggtacatcgtgcactggtacagacagcctccaggcaaggctctggaatggctggctatgatttggggcggaggcagaatcgactacaacagcgccctgaagtccagactgaccatcagcaaggacaacagcaagagccaggtggtgctgaccatgaccaacatggaccctgtggacaccgccacctactactgcgctagaaacttcggcgagaacgccgaggcttactggggacagggaacactggtcaccgtgtctagtgctagcaccaagggcccatccgtcttccccctggcaccctcctccaagagcacctctgggggcacagcggccctgggctgcctggtcaaggactacttccccgaaccggtgacggtgtcgtggaactcaggcgccctgaccagcggcgtgcacaccttcccggctgtcctacagtcctcaggactctactccctcagcagcgtggtgaccgtgccctccagcagcttgggcacccagacctacatctgcaacgtgaatcacaagcccagcaacaccaaggtggacaagagagttgagcccaaatcttgtgacaaaactcacacatgcccaccgtgcccagcacctgaactcctggggggaccgtcagtcttcctcttccccccaaaacccaaggacaccctcatgatctcccggacccctgaggtcacatgcgtggtggtggacgtgagccacgaagaccctgaggtcaagttcaactggtacgtggacggcgtggaggtgcataatgccaagacaaagccgcgggaggagcagtacaacagcacgtaccgtgtggtcagcgtcctcaccgtcctgcaccaggactggctgaatggcaaggagtacaagtgcaaggtctccaacaaagccctcccagcccccatcgagaaaaccatctccaaagccaaagggcagccccgagaaccacaggtgtacaccctgcccccatcccgggaggagatgaccaagaaccaggtcagcctgacctgcctggtcaaaggcttctatcccagcgacatcgccgtggagtgggagagcaatgggcagccggagaacaactacaagaccacgcctcccgtgctggactccgacggctccttcttcctctatagcaagctcaccgtggacaagagcaggtggcagcaggggaacgtcttctcatgctccgtgctgcatgaggctctgcacgcccactacacgcagaagtccctctccctgtctccgggtaaa

SEQ ID NO: 277 - protein, 214 aa, synthetic construct
  REGION 1..214: note = Light chain of h200O1 H1K1 hIgG1 LA
DIQMTQSPSSLSASVGDRVTITCRASQDINIYLNWYQQKPGKVVKLLIYYTSRLHSGVPSRFSGSGSGTDFTLTISSLQPEDVATYFCQQGHTLPYTFGQGTKLEIKRTVAAPSVFIFPPSDEQLKSGTASVVCLLNNFYPREAKVQWKVDNALQSGNSQESVTEQDSKDSTYSLSSTLTLSKADYEKHKVYACEVTHQGLSSPVTKSFNRGEC

SEQ ID NO: 278 - DNA, 645 bp, synthetic construct
  misc_feature 1..645: note = Nucleotide sequence of light chain of h200O1 H1K1 hIgG1 LA
  source 1..645: mol_type = other DNA
gacatccagatgacacagagccctagcagcctgtctgccagcgtgggagacagagtgaccatcacctgtagagccagccaggacatcaacatctacctgaactggtatcagcagaaacccggcaaggtggtcaagctgctgatctactacaccagcagactgcacagcggcgtgccctctagattttctggcagcggctctggcaccgacttcaccctgacaatctctagcctgcagcctgaggacgtggcaacctacttctgccagcaaggccacacactgccctacacatttggccagggcaccaagctggaaatcaagcgaactgtggctgcaccatctgtcttcatcttcccgccatctgatgagcagttgaaatctggaactgcctctgttgtgtgcctgctgaataacttctatcccagagaggccaaagtacagtggaaggtggataacgccctccaatcgggtaactcccaggagagtgtcacagagcaggacagcaaggacagcacctacagcctcagcagcaccctgacgctgagcaaagcagactacgagaaacacaaagtctacgcctgcgaagtcacccatcagggcctgagctcgcccgtcacaaagagcttcaacaggggagagtgttag

SEQ ID NO: 279 - protein, 17 aa, synthetic construct
  REGION 1..17: note = 174J17, h151N5 H4 HCDR3
GRSTMITTTRNYLALDY

SEQ ID NO: 280 - protein, 42 aa, Homo sapiens [sequence omitted]